European Patent Application EP 4 410 971 A1, published August 7, 2024. Title: Mhothd for producing adeno-associated virus, cell and expression vector. Applicant: FUJIFILM Corporation. The sequence listing filed with the application follows.

SEQUENCE LISTING (16 sequences)

SEQ ID NO: 1 - DNA, 7622 bp, synthetic construct
  misc_feature 1..7622: note = plasmid
  source 1..7622: mol_type = other DNA
agcgcccaatacgcaaaccgcctctccccgcgcgttggccgattcattaatgcagctggcacgacaggtttcccgactggaaagcgggcagtgagcgcaacgcaattaatgtgagttagctcactcattaggcaccccaggctttacactttatgcttccggctcgtatgttgtgtggaattgtgagcggataacaatttcacacaggaaacagctatgaccatgattacgaattgcctgcaggcagctgcgcgctcgctcgctcactgaggccgcccgggcaaagcccgggcgtcgggcgacctttggtcgcccggcctcagtgagcgagcgagcgcgcagagagggagtggccaactccatcactaggggttcctatcgatatcaagctttaatagtaatcaattacggggtcattagttcatagcccatatatggagttccgcgttacataacttacggtaaatggcccgcctggctgaccgcccaacgacccccgcccattgacgtcaataatgacgtatgttcccatagtaacgccaatagggactttccattgacgtcaatgggtggagtatttacggtaaactgcccacttggcagtacatcaagtgtatcatatgccaagtacgccccctattgacgtcaatgacggtaaatggcccgcctggcattatgcccagtacatgaccttatgggactttcctacttggcagtacatctacgtattagtcatcgctattaccatggtgatgcggttttggcagtacatcaatgggcgtggatagcggtttgactcacggggatttccaagtctccaccccattgacgtcaatgggagtttgttttggcaccaaaatcaacgggactttccaaaatgtcgtaacaactccgccccattgacgcaaatgggcggtaggcgtgtacggtgggaggtctatataagcagagctggtttagtggatatccttaagggcccagccggcctcgcgagaattctctagaacgccgccatgaccatgattacggattcactggccgtcgttttacaacgtcgtgactgggaaaaccctggcgttacccaacttaatcgccttgcagcacatccccctttcgccagctggcgtaatagcgaagaggcccgcaccgatcgcccttcccaacagttgcgcagcctgaatggcgaatggcgctttgcctggtttccggcaccagaagcggtgccggaaagctggctggagtgcgatcttcctgaggccgatactgtcgtcgtcccctcaaactggcagatgcacggttacgatgcgcccatctacaccaacgtgacctatcccattacggtcaatccgccgtttgttcccacggagaatccgacgggttgttactcgctcacatttaatgttgatgaaagctggctacaggaaggccagacgcgaattatttttgatggcgttaactcggcgtttcatctgtggtgcaacgggcgctgggtcggttacggccaggacagtcgtttgccgtctgaatttgacctgagcgcatttttacgcgccggagaaaaccgcctcgcggtgatggtgctgcgctggagtgacggcagttatctggaagatcaggatatgtggcggatgagcggcattttccgtgacgtctcgttgctgcataaaccgactacacaaatcagcgatttccatgttgccactcgctttaatgatgatttcagccgcgctgtactggaggctgaagttcagatgtgcggcgagttgcgtgactacctacgggtaacagtttctttatggcagggtgaaacgcaggtcgccagcggcaccgcgcctttcggcggtgaaattatcgatgagcgtggtggttatgccgatcgcgtcacactacgtctgaacgtcgaaaacccgaaactgtggagcgccgaaatcccgaatctctatcgtgcggtggttgaactgcacaccgccgacggcacgctgattgaagcagaagcctgcgatgtcggtttccgcgaggtgcggattgaaaatggtctgctgctgctgaacggcaagccgttgctgattcgaggcgttaaccgtcacgagcatcatcctctgcatggtcaggtcatggatgagcagacgatggtgcaggatatcctgctgatgaagcagaacaactttaacgccgtgcgctgttcgcattatccgaaccatccgctgtggtacacgctgtgcgaccgctacggcctgtatgtggtggatgaagccaatattgaaacccacggcatggtgccaatgaatcgtctgaccgatgatccgcgctggctaccggcgatgagcgaacgcgtaacgcgaatggtgcagcgcgatcgtaatcacccgagtgtgatcatctggtcgctggggaatgaatcaggccacggcgctaatcacgacgcgctgtatcgctggatcaaatctgtcgatccttcccgcccggtgcagtatgaaggcggcggagccgacaccacggccaccgatattatttgcccgatgtacgcgcgcgtggatgaagaccagcccttcccggctgtgccgaaatggtccatcaaaaaatggctttcgctacctggagagacgcgcccgctgatcctttgcgaatacgcccacgcgatgggtaacagtcttggcggtttcgctaaatactggcaggcgtttcgtcagtatccccgtttacagggcggcttcgtctgggactgggtggatcagtcgctgattaaatatgatgaaaacggcaacccgtggtcggcttacggcggtgattttggcgatacgccgaacgatcgccagttctgtatgaacggtctggtctttgccgaccgcacgccgcatccagcgctgacggaagcaaaacaccagcagcagtttttccagttccgtttatccgggcaaaccatcgaagtgaccagcgaatacctgttccgtcatagcgataacgagctcctgcactggatggtggcgctggatggtaagccgctggcaagcggtgaagtgcctctggatgtcgctccacaaggtaaacagttgattgaactgcctgaactaccgcagccggagagcgccgggcaactctggctcacagtacgcgtagtgcaaccgaacgcgaccgcatggtcagaagccgggcacatcagcgcctggcagcagtggcgtctggcggaaaacctcagtgtgacgctccccgccgcgtcccacgccatcccgcatctgaccaccagcgaaatggatttttgcatcgagctgggtaataagcgttggcaatttaaccgccagtcaggctttctttcacagatgtggattggcgataaaaaacaactgctgacgccgctgcgcgatcagttcacccgtgcaccgctggataacgacattggcgtaagtgaagcgacccgcattgaccctaacgcctgggtcgaacgctggaaggcggcgggccattaccaggccgaagcagcgttgttgcagtgcacggcagatacacttgctgatgcggtgctgattacgaccgctcacgcgtggcagcatcaggggaaaaccttatttatcagccggaaaacctaccggattgatggtagtggtcaaatggcgattaccgttgatgttgaagtggcgagcgatacaccgcatccggcgcggattggcctgaactgccagctggcgcaggtagcagagcgggtaaactggctcggattagggccgcaagaaaactatcccgaccgccttactgccgcctgttttgaccgctgggatctgccattgtcagacatgtataccccgtacgtcttcccgagcgaaaacggtctgcgctgcgggacgcgcgaattgaattatggcccacaccagtggcgcggcgacttccagttcaacatcagccgctacagtcaacagcaactgatggaaaccagccatcgccatctgctgcacgcggaagaaggcacatggctgaatatcgacggtttccatatggggattggtggcgacgactcctggagcccgtcagtatcggcggaattccagctgagcgccggtcgctaccattaccagttggtctggtgtcaaaaataaagctgacactagtgcggatccacgggtggcatccctgtgacccctccccagtgcctctcctggccctggaagttgccactccagtgcccaccagccttgtcctaataaaattaagttgcatcattttgtctgactaggtgtccttctataatattatggggtggaggggggtggtatggagcaaggggcaagttgggaagacaacctgtagggcctgcggggtctattgggaaccaagctggagtgcagtggcacaatcttggctcactgcaatctccgcctcctgggttcaagcgattctcctgcctcagcctcccgagttgttgggattccaggcatgcatgaccaggctcagctaatttttgtttttttggtagagacggggtttcaccatattggccaggctggtctccaactcctaatctcaggtgatctacccaccttggcctcccaaattgctgggattacaggcgtgaaccactgctcccttccctgtccttatcgatagatctaggaacccctagtgatggagttggccactccctctctgcgcgctcgctcgctcactgaggccgggcgaccaaaggtcgcccgacgcccgggctttgcccgggcggcctcagtgagcgagcgagcgcgcagctgcctgcaggcagcttggcactggccgtcgttttacaacgtcgtgactgggaaaaccctggcgttacccaacttaatcgccttgcagcacatccccctttcgccagctggcgtaatagcgaagaggcccgcaccgatcgcccttcccaacagttgcgcagcctgaatggcgaatggcgcctgatgcggtattttctccttacgcatctgtgcggtatttcacaccgcatacgtcaaagcaaccatagtacgcgccctgtagcggcgcattaagcgcggcgggtgtggtggttacgcgcagcgtgaccgctacacttgccagcgccctagcgcccgctcctttcgctttcttcccttcctttctcgccacgttcgccggctttccccgtcaagctctaaatcgggggctccctttagggttccgatttagtgctttacggcacctcgaccccaaaaaacttgatttgggtgatggttcacgtagtgggccatcgccctgatagacggtttttcgccctttgacgttggagtccacgttctttaatagtggactcttgttccaaactggaacaacactcaaccctatctcgggctattcttttgatttataagggattttgccgatttcggcctattggttaaaaaatgagctgatttaacaaaaatttaacgcgaattttaacaaaatattaacgtttacaattttatggtgcactctcagtacaatctgctctgatgccgcatagttaagccagccccgacacccgccaacacccgctgacgcgccctgacgggcttgtctgctcccggcatccgcttacagacaagctgtgaccgtctccgggagctgcatgtgtcagaggttttcaccgtcatcaccgaaacgcgcgagacgaaagggcctcgtgatacgcctatttttataggttaatgtcatgataataatggtttcttagacgtcaggtggcacttttcggggaaatgtgcgcggaacccctatttgtttatttttctaaatacattcaaatatgtatccgctcatgagacaataaccctgataaatgcttcaataatattgaaaaaggaagagtatgagtattcaacatttccgtgtcgcccttattcccttttttgcggcattttgccttcctgtttttgctcacccagaaacgctggtgaaagtaaaagatgctgaagatcagttgggtgcacgagtgggttacatcgaactggatctcaacagcggtaagatccttgagagttttcgccccgaagaacgttttccaatgatgagcacttttaaagttctgctatgtggcgcggtattatcccgtattgacgccgggcaagagcaactcggtcgccgcatacactattctcagaatgacttggttgagtactcaccagtcacagaaaagcatcttacggatggcatgacagtaagagaattatgcagtgctgccataaccatgagtgataacactgcggccaacttacttctgacaacgatcggaggaccgaaggagctaaccgcttttttgcacaacatgggggatcatgtaactcgccttgatcgttgggaaccggagctgaatgaagccataccaaacgacgagcgtgacaccacgatgcctgtagcaatggcaacaacgttgcgcaaactattaactggcgaactacttactctagcttcccggcaacaattaatagactggatggaggcggataaagttgcaggaccacttctgcgctcggcccttccggctggctggtttattgctgataaatctggagccggtgagcgtgggtctcgcggtatcattgcagcactggggccagatggtaagccctcccgtatcgtagttatctacacgacggggagtcaggcaactatggatgaacgaaatagacagatcgctgagataggtgcctcactgattaagcattggtaactgtcagaccaagtttactcatatatactttagattgatttaaaacttcatttttaatttaaaaggatctaggtgaagatcctttttgataatctcatgaccaaaatcccttaacgtgagttttcgttccactgagcgtcagaccccgtagaaaagatcaaaggatcttcttgagatcctttttttctgcgcgtaatctgctgcttgcaaacaaaaaaaccaccgctaccagcggtggtttgtttgccggatcaagagctaccaactctttttccgaaggtaactggcttcagcagagcgcagataccaaatactgttcttctagtgtagccgtagttaggccaccacttcaagaactctgtagcaccgcctacatacctcgctctgctaatcctgttaccagtggctgctgccagtggcgataagtcgtgtcttaccgggttggactcaagacgatagttaccggataaggcgcagcggtcgggctgaacggggggttcgtgcacacagcccagcttggagcgaacgacctacaccgaactgagatacctacagcgtgagctatgagaaagcgccacgcttcccgaagggagaaaggcggacaggtatccggtaagcggcagggtcggaacaggagagcgcacgagggagcttccagggggaaacgcctggtatctttatagtcctgtcgggtttcgccacctctgacttgagcgtcgatttttgtgatgctcgtcaggggggcggagcctatggaaaaacgccagcaacgcggcctttttacggttcctggccttttgctggccttttgctcacatgttctttcctgcgttatcccctgattctgtggataaccgtattaccgcctttgagtgagctgataccgctcgccgcagccgaacgaccgagcgcagcgagtcagtgagcgaggaagcggaag

SEQ ID NO: 2 - DNA, 7294 bp, synthetic construct
  misc_feature 1..7294: note = plasmid
  source 1..7294: mol_type = other DNA
gcgcgccgatatcgttaacgccccgcgccggccgctctagaactagtggatcccccggaagatcagaagttcctattccgaagttcctattctctagaaagtataggaacttctgatctgcgcagccgccatgccggggttttacgagattgtgattaaggtccccagcgaccttgacgagcatctgcccggcatttctgacagctttgtgaactgggtggccgagaaggaatgggagttgccgccagattctgacatggatctgaatctgattgagcaggcacccctgaccgtggccgagaagctgcagcgcgactttctgacggaatggcgccgtgtgagtaaggccccggaggcccttttctttgtgcaatttgagaagggagagagctacttccacatgcacgtgctcgtggaaaccaccggggtgaaatccatggttttgggacgtttcctgagtcagattcgcgaaaaactgattcagagaatttaccgcgggatcgagccgactttgccaaactggttcgcggtcacaaagaccagaaatggcgccggaggcgggaacaaggtggtggatgagtgctacatccccaattacttgctccccaaaacccagcctgagctccagtgggcgtggactaatatggaacagtatttaagcgcctgtttgaatctcacggagcgtaaacggttggtggcgcagcatctgacgcacgtgtcgcagacgcaggagcagaacaaagagaatcagaatcccaattctgatgcgccggtgatcagatcaaaaacttcagccaggtacatggagctggtcgggtggctcgtggacaaggggattacctcggagaagcagtggatccaggaggaccaggcctcatacatctccttcaatgcggcctccaactcgcggtcccaaatcaaggctgccttggacaatgcgggaaagattatgagcctgactaaaaccgcccccgactacctggtgggccagcagcccgtggaggacatttccagcaatcggatttataaaattttggaactaaacgggtacgatccccaatatgcggcttccgtctttctgggatgggccacgaaaaagttcggcaagaggaacaccatctggctgtttgggcctgcaactaccgggaagaccaacatcgcggaggccatagcccacactgtgcccttctacgggtgcgtaaactggaccaatgagaactttcccttcaacgactgtgtcgacaagatggtgatctggtgggaggaggggaagatgaccgccaaggtcgtggagtcggccaaagccattctcggaggaagcaaggtgcgcgtggaccagaaatgcaagtcctcggcccagatagacccgactcccgtgatcgtcacctccaacaccaacatgtgcgccgtgattgacgggaactcaacgaccttcgaacaccagcagccgttgcaagaccggatgttcaaatttgaactcacccgccgtctggatcatgactttgggaaggtcaccaagcaggaagtcaaagactttttccggtgggcaaaggatcacgtggttgaggtggagcatgaattctacgtcaaaaagggtggagccaagaaaagacccgcccccagtgacgcagatataagtgagcccaaacgggtgcgcgagtcagttgcgcagccatcgacgtcagacgcggaagcttcgatcaactacgcagacaggtaccaaaacaaatgttctcgtcacgtgggcatgaatctgatgctgtttccctgcagacaatgcgagagaatgaatcagaattcaaatatctgcttcactcacggacagaaagactgtttagagtgctttcccgtgtcagaatctcaacccgtttctgtcgtcaaaaaggcgtatcagaaactgtgctacattcatcatatcatgggaaaggtgccagacgcttgcactgcctgcgatctggtcaatgtggatttggatgactgcatctttgaacaataaatgatttaaatcaggtatgtcttttgttgatcaccctccagattggttggaagaagttggtgaaggtcttcgcgagtttttgggccttgaagcgggcccaccgaaaccaaaacccaatcagcagcatcaagatcaagcccgtggtcttgtgctgcctggttataactatctcggacccggaaacggtctcgatcgaggagagcctgtcaacagggcagacgaggtcgcgcgagagcacgacatctcgtacaacgagcagcttgaggcgggagacaacccctacctcaagtacaaccacgcggacgccgagtttcaggagaagctcgccgacgacacatccttcgggggaaacctcggaaaggcagtctttcaggccaagaaaagggttctcgaaccttttggcctggttgaagagggtgctaagacggcccctaccggaaagcggatagacgaccactttccaaaaagaaagaaggctcggaccgaagaggactccaagccttccacctcgtcagacgccgaagctggacccagcggatcccagcagctgcaaatcccagcccaaccagcctcaagtttgggagctgatacaatgtctgcgggaggtggcggcccattgggcgacaataaccaaggtgccgatggagtgggcaatgcctcgggagattggcattgcgattccacgtggatgggggacagagtcgtcaccaagtccacccgaacctgggtgctgcccagctacaacaaccaccagtaccgagagatcaaaagcggctccgtcgacggaagcaacgccaacgcctactttggatacagcaccccctgggggtactttgactttaaccgcttccacagccactggagcccccgagactggcaaagactcatcaacaactactggggcttcagaccccggtccctcagagtcaaaatcttcaacattcaagtcaaagaggtcacggtgcaggactccaccaccaccatcgccaacaacctcacctccaccgtccaagtgtttacggacgacgactaccagctgccctacgtcgtcggcaacgggaccgagggatgcctgccggccttccctccgcaggtctttacgctgccgcagtacggttacgcgacgctgaaccgcgacaacacagaaaatcccaccgagaggagcagcttcttctgcctagagtactttcccagcaagatgctgagaacgggcaacaactttgagtttacctacaactttgaggaggtgcccttccactccagcttcgctcccagtcagaacctgttcaagctggccaacccgctggtggaccagtacttgtaccgcttcgtgagcacaaataacactggcggagtccagttcaacaagaacctggccgggagatacgccaacacctacaaaaactggttcccggggcccatgggccgaacccagggctggaacctgggctccggggtcaaccgcgccagtgtcagcgccttcgccacgaccaataggatggagctcgagggcgcgagttaccaggtgcccccgcagccgaacggcatgaccaacaacctccagggcagcaacacctatgccctggagaacactatgatcttcaacagccagccggcgaacccgggcaccaccgccacgtacctcgagggcaacatgctcatcaccagcgagagcgagacgcagccggtgaaccgcgtggcgtacaacgtcggcgggcagatggccaccaacaaccagagctccaccactgcccccgcgaccggcacgtacaacctccaggaaatcgtgcccggcagcgtgtggatggagagggacgtgtacctccaaggacccatctgggccaagatcccagagacgggggcgcactttcacccctctccggccatgggcggattcggactcaaacacccaccgcccatgatgctcatcaagaacacgcctgtgcccggaaatatcaccagcttctcggacgtgcccgtcagcagcttcatcacccagtacagcaccgggcaggtcaccgtggagatggagtgggagctcaagaaggaaaactccaagaggtggaacccagagatccagtacacaaacaactacaacgacccccagtttgtggactttgccccggacagcaccggggaatacagaaccaccagacctatcggaacccgataccttacccgacccctttaattgcttgttaatcaataaaccgtttaattcgtttcagttgaactttggtctctgcgtatttctttcttatctagtttccatggctacgtagataagtagcatggcgggttaatcattaactacagcccgggcgtttaaacagcgggcggaggggtggagtcgtgacgtgaattacgtcatagggttagggaggtcctgtattagaggtcacgtgagtgttttgcgacattttgcgacaccatgtggtctcgctgggggggggggcccgagtgagcacgcagggtctccattttgaagcgggaggtttgaacgagcgctggcgcgctcactggccgtcgttttacaacgtcgtgactgggaaaaccctggcgttacccaacttaatcgccttgcagcacatccccctttcgccagctggcgtaatagcgaagaggcccgcaccgatcgcccttcccaacagttgcgcagcctgaatggcgaatggaaattgtaagcgttaatattttgttaaaattcgcgttaaatttttgttaaatcagctcatttttttaaccaataggccgaaatcggcaaaatcccttataaatcaaaagaatagaccgagatagggttgagtgttgttccagtttggaacaagagtccactattaagaacgtggactccaacgtcaaagggcgaaaaaccgtctatcagggcgatggcccactacgtgaaccatcaccctaatcaagttttttggggtcgaggtgccgtaaagcactaaatcggaaccctaaagggagcccccgatttagagcttgacggggaaagccggcgaacgtggcgagaaaggaagggaagaaagcgaaaggagcgggcgctagggcgctggcaagtgtagcggtcacgctgcgcgtaaccaccacacccgccgcgcttaatgcgccgctacagggcgcgtcaggtggcacttttcggggaaatgtgcgcggaacccctatttgtttatttttctaaatacattcaaatatgtatccgctcatgagacaataaccctgataaatgcttcaataatattgaaaaaggaagagtatgagtattcaacatttccgtgtcgcccttattcccttttttgcggcattttgccttcctgtttttgctcacccagaaacgctggtgaaagtaaaagatgctgaagatcagttgggtgcacgagtgggttacatcgaactggatctcaacagcggtaagatccttgagagttttcgccccgaagaacgttttccaatgatgagcacttttaaagttctgctatgtggcgcggtattatcccgtattgacgccgggcaagagcaactcggtcgccgcatacactattctcagaatgacttggttgagtactcaccagtcacagaaaagcatcttacggatggcatgacagtaagagaattatgcagtgctgccataaccatgagtgataacactgcggccaacttacttctgacaacgatcggaggaccgaaggagctaaccgcttttttgcacaacatgggggatcatgtaactcgccttgatcgttgggaaccggagctgaatgaagccataccaaacgacgagcgtgacaccacgatgcctgtagcaatggcaacaacgttgcgcaaactattaactggcgaactacttactctagcttcccggcaacaattaatagactggatggaggcggataaagttgcaggaccacttctgcgctcggcccttccggctggctggtttattgctgataaatctggagccggtgagcgtgggtctcgcggtatcattgcagcactggggccagatggtaagccctcccgtatcgtagttatctacacgacggggagtcaggcaactatggatgaacgaaatagacagatcgctgagataggtgcctcactgattaagcattggtaactgtcagaccaagtttactcatatatactttagattgatttaaaacttcatttttaatttaaaaggatctaggtgaagatcctttttgataatctcatgaccaaaatcccttaacgtgagttttcgttccactgagcgtcagaccccgtagaaaagatcaaaggatcttcttgagatcctttttttctgcgcgtaatctgctgcttgcaaacaaaaaaaccaccgctaccagcggtggtttgtttgccggatcaagagctaccaactctttttccgaaggtaactggcttcagcagagcgcagataccaaatactgttcttctagtgtagccgtagttaggccaccacttcaagaactctgtagcaccgcctacatacctcgctctgctaatcctgttaccagtggctgctgccagtggcgataagtcgtgtcttaccgggttggactcaagacgatagttaccggataaggcgcagcggtcgggctgaacggggggttcgtgcacacagcccagcttggagcgaacgacctacaccgaactgagatacctacagcgtgagctatgagaaagcgccacgcttcccgaagggagaaaggcggacaggtatccggtaagcggcagggtcggaacaggagagcgcacgagggagcttccagggggaaacgcctggtatctttatagtcctgtcgggtttcgccacctctgacttgagcgtcgatttttgtgatgctcgtcaggggggcggagcctatggaaaaacgccagcaacgcggcctttttacggttcctggccttttgctggccttttgctcacatgttctttcctgcgttatcccctgattctgtggataaccgtattaccgcctttgagtgagctgataccgctcgccgcagccgaacgaccgagcgcagcgagtcagtgagcgaggaagcggaagagcgcccaatacgcaaaccgcctctccccgcgcgttggccgattcattaatgcagctggcacgacaggtttcccgactggaaagcgggcagtgagcgcaacgcaattaatgtgagttagctcactcattaggcaccccaggctttacactttatgcttccggctcgtatgttgtgtggaattgtgagcggataacaatttcacacaggaaacagctatgaccatgattacgccaa

SEQ ID NO: 3 - DNA, 8451 bp, synthetic construct
  misc_feature 1..8451: note = plasmid
  source 1..8451: mol_type = other DNA
ggtacccaactccatgcttaacagtccccaggtacagcccaccctgcgtcgcaaccaggaacagctctacagcttcctggagcgccactcgccctacttccgcagccacagtgcgcagattaggagcgccacttctttttgtcacttgaaaaacatgtaaaaataatgtactaggagacactttcaataaaggcaaatgtttttatttgtacactctcgggtgattatttaccccccacccttgccgtctgcgccgtttaaaaatcaaaggggttctgccgcgcatcgctatgcgccactggcagggacacgttgcgatactggtgtttagtgctccacttaaactcaggcacaaccatccgcggcagctcggtgaagttttcactccacaggctgcgcaccatcaccaacgcgtttagcaggtcgggcgccgatatcttgaagtcgcagttggggcctccgccctgcgcgcgcgagttgcgatacacagggttgcagcactggaacactatcagcgccgggtggtgcacgctggccagcacgctcttgtcggagatcagatccgcgtccaggtcctccgcgttgctcagggcgaacggagtcaactttggtagctgccttcccaaaaagggtgcatgcccaggctttgagttgcactcgcaccgtagtggcatcagaaggtgaccgtgcccggtctgggcgttaggatacagcgcctgcatgaaagccttgatctgcttaaaagccacctgagcctttgcgccttcagagaagaacatgccgcaagacttgccggaaaactgattggccggacaggccgcgtcatgcacgcagcaccttgcgtcggtgttggagatctgcaccacatttcggccccaccggttcttcacgatcttggccttgctagactgctccttcagcgcgcgctgcccgttttcgctcgtcacatccatttcaatcacgtgctccttatttatcataatgctcccgtgtagacacttaagctcgccttcgatctcagcgcagcggtgcagccacaacgcgcagcccgtgggctcgtggtgcttgtaggttacctctgcaaacgactgcaggtacgcctgcaggaatcgccccatcatcgtcacaaaggtcttgttgctggtgaaggtcagctgcaacccgcggtgctcctcgtttagccaggtcttgcatacggccgccagagcttccacttggtcaggcagtagcttgaagtttgcctttagatcgttatccacgtggtacttgtccatcaacgcgcgcgcagcctccatgcccttctcccacgcagacacgatcggcaggctcagcgggtttatcaccgtgctttcactttccgcttcactggactcttccttttcctcttgcgtccgcataccccgcgccactgggtcgtcttcattcagccgccgcaccgtgcgcttacctcccttgccgtgcttgattagcaccggtgggttgctgaaacccaccatttgtagcgccacatcttctctttcttcctcgctgtccacgatcacctctggggatggcgggcgctcgggcttgggagaggggcgcttctttttctttttggacgcaatggccaaatccgccgtcgaggtcgatggccgcgggctgggtgtgcgcggcaccagcgcatcttgtgacgagtcttcttcgtcctcggactcgagacgccgcctcagccgcttttttgggggcgcgcggggaggcggcggcgacggcgacggggacgacacgtcctccatggttggtggacgtcgcgccgcaccgcgtccgcgctcgggggtggtttcgcgctgctcctcttcccgactggccatttccttctcctataggcagaaaaagatcatggagtcagtcgagaaggaggacagcctaaccgccccctttgagttcgccaccaccgcctccaccgatgccgccaacgcgcctaccaccttccccgtcgaggcacccccgcttgaggaggaggaagtgattatcgagcaggacccaggttttgtaagcgaagacgacgaggatcgctcagtaccaacagaggataaaaagcaagaccaggacgacgcagaggcaaacgaggaacaagtcgggcggggggaccaaaggcatggcgactacctagatgtgggagacgacgtgctgttgaagcatctgcagcgccagtgcgccattatctgcgacgcgttgcaagagcgcagcgatgtgcccctcgccatagcggatgtcagccttgcctacgaacgccacctgttctcaccgcgcgtaccccccaaacgccaagaaaacggcacatgcgagcccaacccgcgcctcaacttctaccccgtatttgccgtgccagaggtgcttgccacctatcacatctttttccaaaactgcaagatacccctatcctgccgtgccaaccgcagccgagcggacaagcagctggccttgcggcagggcgctgtcatacctgatatcgcctcgctcgacgaagtgccaaaaatctttgagggtcttggacgcgacgagaaacgcgcggcaaacgctctgcaacaagaaaacagcgaaaatgaaagtcactgtggagtgctggtggaacttgagggtgacaacgcgcgcctagccgtgctgaaacgcagcatcgaggtcacccactttgcctacccggcacttaacctaccccccaaggttatgagcacagtcatgagcgagctgatcgtgcgccgtgcacgacccctggagagggatgcaaacttgcaagaacaaaccgaggagggcctacccgcagttggcgatgagcagctggcgcgctggcttgagacgcgcgagcctgccgacttggaggagcgacgcaagctaatgatggccgcagtgcttgttaccgtggagcttgagtgcatgcagcggttctttgctgacccggagatgcagcgcaagctagaggaaacgttgcactacacctttcgccagggctacgtgcgccaggcctgcaaaatttccaacgtggagctctgcaacctggtctcctaccttggaattttgcacgaaaaccgcctcgggcaaaacgtgcttcattccacgctcaagggcgaggcgcgccgcgactacgtccgcgactgcgtttacttatttctgtgctacacctggcaaacggccatgggcgtgtggcagcaatgcctggaggagcgcaacctaaaggagctgcagaagctgctaaagcaaaacttgaaggacctatggacggccttcaacgagcgctccgtggccgcgcacctggcggacattatcttccccgaacgcctgcttaaaaccctgcaacagggtctgccagacttcaccagtcaaagcatgttgcaaaactttaggaactttatcctagagcgttcaggaattctgcccgccacctgctgtgcgcttcctagcgactttgtgcccattaagtaccgtgaatgccctccgccgctttggggtcactgctaccttctgcagctagccaactaccttgcctaccactccgacatcatggaagacgtgagcggtgacggcctactggagtgtcactgtcgctgcaacctatgcaccccgcaccgctccctggtctgcaattcgcaactgcttagcgaaagtcaaattatcggtacctttgagctgcagggtccctcgcctgacgaaaagtccgcggctccggggttgaaactcactccggggctgtggacgtcggcttaccttcgcaaatttgtacctgaggactaccacgcccacgagattaggttctacgaagaccaatcccgcccgccaaatgcggagcttaccgcctgcgtcattacccagggccacatccttggccaattgcaagccatcaacaaagcccgccaagagtttctgctacgaaagggacggggggtttacctggacccccagtccggcgaggagctcaacccaatccccccgccgccgcagccctatcagcagccgcgggcccttgcttcccaggatggcacccaaaaagaagctgcagctgccgccgccgccacccacggacgaggaggaatactgggacagtcaggcagaggaggttttggacgaggaggaggagatgatggaagactgggacagcctagacgaagcttccgaggccgaagaggtgtcagacgaaacaccgtcaccctcggtcgcattcccctcgccggcgccccagaaattggcaaccgttcccagcatcgctacaacctccgctcctcaggcgccgccggcactgcctgttcgccgacccaaccgtagatgggacaccactggaaccagggccggtaagtctaagcagccgccgccgttagcccaagagcaacaacagcgccaaggctaccgctcgtggcgcgggcacaagaacgccatagttgcttgcttgcaagactgtgggggcaacatctccttcgcccgccgctttcttctctaccatcacggcgtggccttcccccgtaacatcctgcattactaccgtcatctctacagcccctactgcaccggcggcagcggcagcggcagcaacagcagcggtcacacagaagcaaaggcgaccggatagcaagactctgacaaagcccaagaaatccacagcggcggcagcagcaggaggaggagcgctgcgtctggcgcccaacgaacccgtatcgacccgcgagcttagaaataggatttttcccactctgtatgctatatttcaacaaagcaggggccaagaacaagagctgaaaataaaaaacaggtctctgcgctccctcacccgcagctgcctgtatcacaaaagcgaagatcagcttcggcgcacgctggaagacgcggaggctctcttcagcaaatactgcgcgctgactcttaaggactagtttcgcgccctttctcaaatttaagcgcgaaaactacgtcatctccagcggccacacccggcgccagcacctgtcgtcagcgccattatgagcaaggaaattcccacgccctacatgtggagttaccagccacaaatgggacttgcggctggagctgcccaagactactcaacccgaataaactacatgagcgcgggaccccacatgatatcccgggtcaacggaatccgcgcccaccgaaaccgaattctcctcgaacaggcggctattaccaccacacctcgtaataaccttaatccccgtagttggcccgctgccctggtgtaccaggaaagtcccgctcccaccactgtggtacttcccagagacgcccaggccgaagttcagatgactaactcaggggcgcagcttgcgggcggctttcgtcacagggtgcggtcgcccgggcgcggccgcaatcgatgtaggatgttgcccctcctgacgcggtaggagaaggggagggtgccctgcatgtctgccgctgctcttgctcttgccgctgctgaggaggggggcgcatctgccgcagcaccggatgcatctgggaaaagcaaaaaaggggctcgtccctgtttccggaggaatttgcaagcggggtcttgcatgacggggaggcaaacccccgttcgccgcagtccggccggcccgagactcgaaccgggggtcctgcgactcaacccttggaaaataaccctccggctacagggagcgagccacttaatgctttcgctttccagcctaaccgcttacgccgcgcgcggccagtggccaaaaaagctagcgcagcagccgccgcgcctggaaggaagccaaaaggagcgctcccccgttgtctgacgtcgcacacctgggttcgacacgcgggcggtaaccgcatggatcacggcggacggccggatccggggttcgaaccccggtcgtccgccatgatacccttgcgaatttatccaccagaccacggaagagtgcccgcttacaggctctccttttgcacggtctagagcgtcaacgactgcgcacgcctcaccggccagagcgtcccgaccatggagcactttttgccgctgcgcaacatctggaaccgcgtccgcgactttccgcgcgcctccaccaccgccgccggcatcacctggatgtccaggtacatctacggattacgtcgacgtttaaaccatatgatcagctcactcaaaggcggtaatacggttatccacagaatcaggggataacgcaggaaagaacatgtgagcaaaaggccagcaaaaggccaggaaccgtaaaaaggccgcgttgctggcgtttttccataggctccgcccccctgacgagcatcacaaaaatcgacgctcaagtcagaggtggcgaaacccgacaggactataaagataccaggcgtttccccctggaagctccctcgtgcgctctcctgttccgaccctgccgcttaccggatacctgtccgcctttctcccttcgggaagcgtggcgctttctcatagctcacgctgtaggtatctcagttcggtgtaggtcgttcgctccaagctgggctgtgtgcacgaaccccccgttcagcccgaccgctgcgccttatccggtaactatcgtcttgagtccaacccggtaagacacgacttatcgccactggcagcagccactggtaacaggattagcagagcgaggtatgtaggcggtgctacagagttcttgaagtggtggcctaactacggctacactagaagaacagtatttggtatctgcgctctgctgaagccagttaccttcggaaaaagagttggtagctcttgatccggcaaacaaaccaccgctggtagcggtggtttttttgtttgcaagcagcagattacgcgcagaaaaaaaggatctcaagaagatcctttgatcttttctacggggtctgacgctcagtggaacgaaaactcacgttaagggattttggtcatgagattatcaaaaaggatcttcacctagatccttttaaattaaaaatgaagttttaaatcaatctaaagtatatatgagtaaacttggtctgacagttaccaatgcttaatcagtgaggcacctatctcagcgatctgtctatttcgttcatccatagttgcctgactccccgtcgtgtagataactacgatacgggagggcttaccatctggccccagtgctgcaatgataccgcgagacccacgctcaccggctccagatttatcagcaataaaccagccagccggaagggccgagcgcagaagtggtcctgcaactttatccgcctccatccagtctattaattgttgccgggaagctagagtaagtagttcgccagttaatagtttgcgcaacgttgttgccattgctacaggcatcgtggtgtcacgctcgtcgtttggtatggcttcattcagctccggttcccaacgatcaaggcgagttacatgatcccccatgttgtgcaaaaaagcggttagctccttcggtcctccgatcgttgtcagaagtaagttggccgcagtgttatcactcatggttatggcagcactgcataattctcttactgtcatgccatccgtaagatgcttttctgtgactggtgagtactcaaccaagtcattctgagaatagtgtatgcggcgaccgagttgctcttgcccggcgtcaatacgggataataccgcgccacatagcagaactttaaaagtgctcatcattggaaaacgttcttcggggcgaaaactctcaaggatcttaccgctgttgagatccagttcgatgtaacccactcgtgcacccaactgatcttcagcatcttttactttcaccagcgtttctgggtgagcaaaaacaggaaggcaaaatgccgcaaaaaagggaataagggcgacacggaaatgttgaatactcatactcttcctttttcaatattattgaagcatttatcagggttattgtctcatgagcggatacatatttgaatgtatttagaaaaataaacaaataggggttccgcgcacatttccccgaaaagtgccacctaaattgtaagcgttaatattttgttaaaattcgcgttaaatttttgttaaatcagctcattttttaaccaataggccgaaatcggcaaaatcccttataaatcaaaagaatagaccgagatagggttgagtgttgttccagtttggaacaagagtccactattaaagaacgtggactccaacgtcaaagggcgaaaaaccgtctatcagggcgatggcccactacgtgaaccatcaccctaatcaagttttttggggtcgaggtgccgtaaagcactaaatcggaaccctaaagggagcccccgatttagagcttgacggggaaagccggcgaacgtggcgagaaaggaagggaagaaagcgaaaggagcgggcgctagggcgctggcaagtgtagcggtcacgctgcgcgtaaccaccacacccgccgcgcttaatgcgccgctacagggcgcgatggatcc

SEQ ID NO: 4 - DNA, 4586 bp, synthetic construct
  misc_feature 1..4586: note = plasmid
  source 1..4586: mol_type = other DNA
tcgcgcgtttcggtgatgacggtgaaaacctctgacacatgcagctcccggagactgtcacagcttgtctgtaagcggatgccgggagcagacaagcccgtcagggcgcgtcagcgggtgttggcgggtgtcggggctggcttaactatgcggcatcagagcagattgtactgagagtgcaccatatgcggtgtgaaataccgcacagatgcgtaaggagaaaataccgcatcaggcgccattcgccattcaggctgcgcaactgttgggaagggcgatcggtgcgggcctcttcgctattacgccagctggcgaaagggggatgtgctgcaaggcgattaagttgggtaacgccagggttttcccagtcacgacgttgtaaaacgacggccagtgaattgacgcgtattgggatgacattgattattgactagttattaatagtaatcaattacggggtcattagttcatagcccatatatggagttccgcgttacataacttacggtaaatggcccgcctggctgaccgcccaacgacccccgcccattgacgtcaataatgacgtatgttcccatagtaacgccaatagggactttccattgacgtcaatgggtggagtatttacggtaaactgcccacttggcagtacatcaagtgtatcatatgccaagtacgccccctattgacgtcaatgacggtaaatggcccgcctggcattatgcccagtacatgaccttatgggactttcctacttggcagtacatctacgtattagtcatcgctattaccatggtgatgcggttttggcagtacatcaatgggcgtggatagcggtttgactcacggggatttccaagtctccaccccattgacgtcaatgggagtttgttttggaaccaaaatcaacgggactttccaaaatgtcgtaacaactccgccccattgacgcaaatgggcggtaggcgtgtacggtgggaggtctatataagcagagctctccctatcagtgatagagatctccctatcagtgatagagatcgtcgacgagctcgtttagtgaaccgtcagatcgcctggagacgccatccacgctgttttgacctccatagaagacaccgggaccgatccagcctccggactctagcgtttaaacttaagcttgccaccatgactacgtccggcgttccatttggcatgacactacgaccaacacgatctcggttgtctcggcgcactccgtacagtagggatcgcctacctccttttgagacagagacccgcgctaccatactggaggatcatccgctgctgcccgaatgtaacactttgacaatgcacaacgtgagttacgtgcgaggtcttccctgcagtgtgggatttacgctgattcaggaatgggttgttccctgggatatggttctgacgcgggaggagcttgtaatcctgaggaagtgtatgcacgtgtgcctgtgttgtgccaacattgatatcatgacgagcatgatgatccatggttacgagtcctgggctctccactgtcattgttccagtcccggttccctgcagtgcatagccggcgggcaggttttggccagctggtttaggatggtggtggatggcgccatgtttaatcagaggtttatatggtaccgggaggtggtgaattacaacatgccaaaagaggtaatgtttatgtccagcgtgtttatgaggggtcgccacttaatctacctgcgcttgtggtatgatggccacgtgggttctgtggtccccgccatgagctttggatacagcgccttgcactgtgggattttgaacaatattgtggtgctgtgctgcagttactgtgctgatttaagtgagatcagggtgcgctgctgtgcccggaggacaaggcgtctcatgctgcgggcggtgcgaatcatcgctgaggagaccactgccatgttgtattcctgcaggacggagcggcggcggcagcagtttattcgcgcgctgctgcagcaccaccgccctatcctgatgcacgattatgactctacccccatgtaggcggccgctcgagtctagagggcccgtttaaacccgctgatcagcctcgactgtgccttctagttgccagccatctgttgtttgcccctcccccgtgccttccttgaccctggaaggtgccactcccactgtcctttcctaataaaatgaggaaattgcatcgcattgtctgagtaggtgtcattctattctggggggtggggtggggcaggacagcaagggggaggattgggaagacaatagcaggcatgctggggatgcggtgggctctatggatcccaatggcgcgccgagcttggcgtaatcatggtcatagctgtttcctgtgtgaaattgttatccgctcacaattccacacaacatacgagccggaagcataaagtgtaaagcctggggtgcctaatgagtgagctaactcacattaattgcgttgcgctcactgcccgctttccagtcgggaaacctgtcgtgccagctgcattaatgaatcggccaacgcgcggggagaggcggtttgcgtattgggcgctgttccgcttcctcgctcactgactcgctgcgctcggtcgttcggctgcggcgagcggtatcagctcactcaaaggcggtaatacggttatccacagaatcaggggataacgcaggaaagaacatgtgagcaaaaggccagcaaaaggccaggaaccgtaaaaaggccgcgttgctggcgtttttccataggctccgcccccctgacgagcatcacaaaaatcgacgctcaagtcagaggtggcgaaacccgacaggactataaagataccaggcgtttccccctggaagctccctcgtgcgctctcctgttccgaccctgccgcttaccggatacctgtccgcctttctcccttcgggaagcgtggcgctttctcatagctcacgctgtaggtatctcagttcggtgtaggtcgttcgctccaagctgggctgtgtgcacgaaccccccgttcagcccgaccgctgcgccttatccggtaactatcgtcttgagtccaacccggtaagacacgacttatcgccactggcagcagccactggtaacaggattagcagagcgaggtatgtaggcggtgctacagagttcttgaagtggtggcctaactacggctacactagaagaacagtatttggtatctgcgctctgctgaagccagttaccttcggaaaaagagttggtagctcttgatccggcaaacaaaccaccgctggtagcggtggtttttttgtttgcaagcagcagattacgcgcagaaaaaaaggatctcaagaagatcctttgatcttttctacggggtctgacgctcagtggaacgaaaactcacgttaagggattttggtcatgagattatcaaaaaggatcttcacctagatccttttaaattaaaaatgaagttttaaatcaatctaaagtatatatgagtaaacttggtctgacagttaccaatgcttaatcagtgaggcacctatctcagcgatctgtctatttcgttcatccatagttgcctgactccccgtcgtgtagataactacgatacgggagggcttaccatctggccccagtgctgcaatgataccgcgagaaccacgctcaccggctccagatttatcagcaataaaccagccagccggaagggccgagcgcagaagtggtcctgcaactttatccgcctccatccagtctattaattgttgccgggaagctagagtaagtagttcgccagttaatagtttgcgcaacgttgttgccattgctacaggcatcgtggtgtcacgctcgtcgtttggtatggcttcattcagctccggttcccaacgatcaaggcgagttacatgatcccccatgttgtgcaaaaaagcggttagctccttcggtcctccgatcgttgtcagaagtaagttggccgcagtgttatcactcatggttatggcagcactgcataattctcttactgtcatgccatccgtaagatgcttttctgtgactggtgagtactcaaccaagtcattctgagaatagtgtatgcggcgaccgagttgctcttgcccggcgtcaatacgggataataccgcgccacatagcagaactttaaaagtgctcatcattggaaaacgttcttcggggcgaaaactctcaaggatcttaccgctgttgagatccagttcgatgtaacccactcgtgcacccaactgatcttcagcatcttttactttcaccagcgtttctgggtgagcaaaaacaggaaggcaaaatgccgcaaaaaagggaataagggcgacacggaaatgttgaatactcatactcttcctttttcaatattattgaagcatttatcagggttattgtctcatgagcggatacatatttgaatgtatttagaaaaataaacaaataggggttccgcgcacatttccccgaaaagtgccacctgacgtctaagaaaccattattatcatgacattaacctataaaaataggcgtatcacgaggcccttttgtc

SEQ ID NO: 5 - DNA, 5872 bp, synthetic construct
  misc_feature 1..5872: note = plasmid
  source 1..5872: mol_type = other DNA
tcgcgcgtttcggtgatgacggtgaaaacctctgacacatgcagctcccggagactgtcacagcttgtctgtaagcggatgccgggagcagacaagcccgtcagggcgcgtcagcgggtgttggcgggtgtcggggctggcttaactatgcggcatcagagcagattgtactgagagtgcaccatatgcggtgtgaaataccgcacagatgcgtaaggagaaaataccgcatcaggcgccattcgccattcaggctgcgcaactgttgggaagggcgatcggtgcgggcctcttcgctattacgccagctggcgaaagggggatgtgctgcaaggcgattaagttgggtaacgccagggttttcccagtcacgacgttgtaaaacgacggccagtgaattgacgcgtattgggatggttttagggcggagtaacttgtatgtgttgggaattgtagttttcttaaaatgggaagtgacgtaacgtgggaaaacggaagtgacgatttgaggaagttgtgggttttttggctttcgtttctgggcgtaggttcgcgtgcggttttctgggtgttttttgtggactttaaccgttacgtcattttttagtcctatatatactcgctctgcacttggcccttttttacactgtgactgattgagctggtgccgtgtcgagtggtgtttttttaataggttttcttttttactggtaaggctgactgttatggctgccgctgtggaagcgctgtatgttgttctggagcgggagggtgctattttgcctaggcaggagggtttttcaggtgtttatgtgtttttctctcctattaattttgttatacctcctatgggggctgtaatgttgtctctacgcctgcgggtatgtattcccccgggctatttcggtcgctttttagcactgaccgatgtgaatcaacctgatgtgtttaccgagtcttacattatgactccggacatgaccgaggagctgtcggtggtgctttttaatcacggtgaccagtttttttacggtcacgccggcatggccgtagtccgtcttatgcttataagggttgtttttcctgttgtaagacaggcttctaatgtttaaatgtttttttgttattttattttgtgtttatgcagaaacccgcagacatgtttgagagaaaaatggtgtctttttctgtggtggttccggagcttacctgcctttatctgcatgagcatgactacgatgtgctttcttttttgcgcgaggctttgcctgattttttgagcagcaccttgcattttatatcgccgcccatgcaacaagcttacatcggggctacgctggttagcatagctccgagtatgcgtgtcataatcagtgtgggttcttttgtcatggttcctggcggggaagtggccgcgctggtccgtgcagacctgcacgattatgttcagctggccctgcgaagggacctacgggatcgcggtatttttgttaatgttccgcttttgaatcttatacaggtctgtgaggaacctgaatttttgcaatcatgattcgctgcttgaggctgaaggtggagggcgctctggagcagatttttacaatggccggacttaatattcgggatttgcttagagatatattgagaaggtggcgagatgagaattatttgggcatggttgaaggtgctggaatgtttatagaggagattcaccctgaagggtttagcctttacgtccacttggacgtgagggccgtttgccttttggaagccattgtgcaacatcttacaaatgccattatctgttctttggctgtagagtttgaccacgccaccggaggggagcgcgttcacttaatagatcttcattttgaggttttggataatcttttggaataaaaaaaaaaaacatggttcttccagctcttcccgctcctcccgtgtgtgactcgcagaacgaatgtgtaggttggctgggtgtggcttattctgcggtggtggatgttatcagggcagcggcgcatgaaggagtttacatagaacccgaagccagggggcgcctggatgctttgagagagtggatatactacaactactacacagagcgatctaagcggcgagaccggagacgcagatctgtttgtcacgcccgcacctggttttgcttcaggaaatatgactacgtccggcgttccatttggcatgacactacgaccaacacgatctcggttgtctcggcgcactccgtacagtagggatcgtctacctccttttgagacagaaacccgcgctaccatactggaggatcatccgctgctgcccgaatgtaacactttgacaatgcacaacgtgagttacgtgcgaggtcttccctgcagtgtgggatttacgctgattcaggaatgggttgttccctgggatatggttctaacgcgggaggagcttgtaatcctgaggaagtgtatgcacgtgtgcctgtgttgtgccaacattgatatcatgacgagcatgatgatccatggttacgagtcctgggctctccactgtcattgttccagtcccggttccctgcagtgtatagccggcgggcaggttttggccagctggtttaggatggtggtggatggcgccatgtttaatcagaggtttatatggtaccgggaggtggtgaattacaacatgccaaaagaggtaatgtttatgtccagcgtgtttatgaggggtcgccacttaatctacctgcgcttgtggtatgatggccacgtgggttctgtggtccccgccatgagctttggatacagcgccttgcactgtgggattttgaacaatattgtggtgctgtgctgcagttactgtgctgatttaagtgagatcagggtgcgctgctgtgcccggaggacaaggcgccttatgctgcgggcggtgcgaatcatcgctgaggagaccactgccatgttgtattcctgcaggacggagcggcggcggcagcagtttattcgcgcgctgctgcagcaccaccgccctatcctgatgcacgattatgactctacccccatgtaggcgtggacttctccttcgccgcccgttaagcaaccgcaagttggacagcagcctgtggctcagcagctggacagcgacatgaacttaagtgagctgcccggggagtttattaatatcactgatgagcgtttggctcgacaggaaaccgtgtggaatataacacctaagaatatgtctgttacccatgatatgatgctttttaaggccagccggggagaaaggactgtgtactctgtgtgttgggagggaggtggcaggttgaatactagggttctgtgagtttgattaaggtacggtgatctgtataagctatgtggtggtggggctatactactgaatgaaaaatgacttgaaattttctgcaattgaaaaataaacacgttgaaacataacacaaacgattctttattcttgggcaatgtatgaaaaagtgtaagaggatgtggcaaatatttcattaatgtagttgtggccagaccagtcccatgaaaatgacatagagtatgcacttggagttgtgtctcctgtttcctgtgtaccgtttagtgtaatggttatcccaatggcgcgccgagcttggcgtaatcatggtcatagctgtttcctgtgtgaaattgttatccgctcacaattccacacaacatacgagccggaagcataaagtgtaaagcctggggtgcctaatgagtgagctaactcacattaattgcgttgcgctcactgcccgctttccagtcgggaaacctgtcgtgccagctgcattaatgaatcggccaacgcgcggggagaggcggtttgcgtattgggcgctgttccgcttcctcgctcactgactcgctgcgctcggtcgttcggctgcggcgagcggtatcagctcactcaaaggcggtaatacggttatccacagaatcaggggataacgcaggaaagaacatgtgagcaaaaggccagcaaaaggccaggaaccgtaaaaaggccgcgttgctggcgtttttccataggctccgcccccctgacgagcatcacaaaaatcgacgctcaagtcagaggtggcgaaacccgacaggactataaagataccaggcgtttccccctggaagctccctcgtgcgctctcctgttccgaccctgccgcttaccggatacctgtccgcctttctcccttcgggaagcgtggcgctttctcatagctcacgctgtaggtatctcagttcggtgtaggtcgttcgctccaagctgggctgtgtgcacgaaccccccgttcagcccgaccgctgcgccttatccggtaactatcgtcttgagtccaacccggtaagacacgacttatcgccactggcagcagccactggtaacaggattagcagagcgaggtatgtaggcggtgctacagagttcttgaagtggtggcctaactacggctacactagaagaacagtatttggtatctgcgctctgctgaagccagttaccttcggaaaaagagttggtagctcttgatccggcaaacaaaccaccgctggtagcggtggtttttttgtttgcaagcagcagattacgcgcagaaaaaaaggatctcaagaagatcctttgatcttttctacggggtctgacgctcagtggaacgaaaactcacgttaagggattttggtcatgagattatcaaaaaggatcttcacctagatccttttaaattaaaaatgaagttttaaatcaatctaaagtatatatgagtaaacttggtctgacagttaccaatgcttaatcagtgaggcacctatctcagcgatctgtctatttcgttcatccatagttgcctgactccccgtcgtgtagataactacgatacgggagggcttaccatctggccccagtgctgcaatgataccgcgagaaccacgctcaccggctccagatttatcagcaataaaccagccagccggaagggccgagcgcagaagtggtcctgcaactttatccgcctccatccagtctattaattgttgccgggaagctagagtaagtagttcgccagttaatagtttgcgcaacgttgttgccattgctacaggcatcgtggtgtcacgctcgtcgtttggtatggcttcattcagctccggttcccaacgatcaaggcgagttacatgatcccccatgttgtgcaaaaaagcggttagctccttcggtcctccgatcgttgtcagaagtaagttggccgcagtgttatcactcatggttatggcagcactgcataattctcttactgtcatgccatccgtaagatgcttttctgtgactggtgagtactcaaccaagtcattctgagaatagtgtatgcggcgaccgagttgctcttgcccggcgtcaatacgggataataccgcgccacatagcagaactttaaaagtgctcatcattggaaaacgttcttcggggcgaaaactctcaaggatcttaccgctgttgagatccagttcgatgtaacccactcgtgcacccaactgatcttcagcatcttttactttcaccagcgtttctgggtgagcaaaaacaggaaggcaaaatgccgcaaaaaagggaataagggcgacacggaaatgttgaatactcatactcttcctttttcaatattattgaagcatttatcagggttattgtctcatgagcggatacatatttgaatgtatttagaaaaataaacaaataggggttccgcgcacatttccccgaaaagtgccacctgacgtctaagaaaccattattatcatgacattaacctataaaaataggcgtatcacgaggcccttttgtc

SEQ ID NO: 6 - DNA, 11039 bp, synthetic construct
  misc_feature 1..11039: note = plasmid
  source 1..11039: mol_type = other DNA
ttgagatcctttttttctgcgcgtaatctgctgcttgcaaacaaaaaaaccaccgctaccagcggtggtttgtttgccggatcaagagctaccaactctttttccgaaggtaactggcttcagcagagcgcagataccaaatactgtccttctagtgtagccgtagttaggccaccacttcaagaactctgtagcaccgcctacatacctcgctctgctaatcctgttaccagtggctgctgccagtggcgataagtcgtgtcttaccgggttggactcaagacgatagttaccggataaggcgcagcggtcgggctgaacggggggttcgtgcacacagcccagcttggagcgaacgacctacaccgaactgagatacctacagcgtgagctatgagaaagcgccacgcttcccgaagggagaaaggcggacaggtatccggtaagcggcagggtcggaacaggagagcgcacgagggagcttccagggggaaacgcctggtatctttatagtcctgtcgggtttcgccacctctgacttgagcgtcgatttttgtgatgctcgtcaggggggcggagcctatggaaaaacgccagcaacgcggcctttttacggttcctggccttttgctggccttttgctcacatgttctttcctgcgttatcccctgattctgtggataaccgtattaccgccatgcatagatctaaatgagtcttcggacctcgcgggggccgcttaagcggtggttagggtttgtctgacgcggggggagggggaaggaacgaaacactctcattcggaggcggctcggggtttggtcttggtggccacgggcacgcagaagagcgccgcgatcctcttaagcacccccccgccctccgtggaggcgggggtttggtcggcgggtggtaactggcgggccgctgactcgggcgggtcgcgcgccccagagtgtgaccttttcggtctgctcgcagacccccgggcggcgccgccgcggcggcgacgggctcgctgggtcctaggctccatggggaccgtatacgtggacaggctctggagcatccgcacgactgcggtgatattaccggagaccttctgcgggacgagccgggtcacgcggctgacgcggagcgtccgttgggcgacaaacaccaggacggggcacaggtacactatcttgtcacccggaggcgcgagggactgcaggagcttcagggagtggcgcagctgcttcatccccgtggcccgttgctcgcgtttgctggcggtgtccccggaagaaatatatttgcatgtctttagttctatgatgacacaaaccccgcccagcgtcttgtcattggcgaattcgaacacgcagatgcagtcggggcggcgcggtcccaggtccacttcgcatattaaggtgacgcgtgtggcctcgaacaccgagcgaccctgcagcgacccgcttaaaagcttgattcttctgacacaacagtctcgaacttaagctgcagaagttggtcgtgaggcactgggcaggtaagtatcaaggttacaagacaggtttaaggagaccaatagaaactgggcttgtcgagacagagaagactcttgcgtttctgataggcacctattggtcttactgacatccactttgcctttctctccacaggtgtccactcccagttcaattacagctcttaaggctagagtacttaatacgactcactataggctagcctggcttgaggctcaggacgcaaatcttgaggatgttcagcgggagttttccgggctgcgagtaattggtgatgaggacgaggatggttcggaggatggggaattttcagacctggatctgtctgacagcgaccatgaaggggatgagggtgggggggctgttggagggggcaggagtctgcactccctgtattcactgagcgtcgtctaataaagatgtctattgatctcttttagtgtgaatcatgtctgacgaggggccaggtacaggacctggaaatggcctaggagagaagggagacacatctggaccagaaggctccggcggcagtggacctcaaagaagagggggtgataaccatggacgaggacggggaagaggacgaggacgaggaggcggaagaccaggagccccgggcggctcaggatcagggccaagacatagagatggtgtccggagaccccaaaaacgtccaagttgcattggctgcaaagggacccacggtggaacaggagcaggagcaggagcgggaggggcaggagcaggaggggcaggagcaggaggaggggcaggagcaggaggaggggcaggaggggcaggaggggcaggaggggcaggagcaggaggaggggcaggagcaggaggaggggcaggaggggcaggaggggcaggagcaggaggaggggcaggagcaggaggaggggcaggaggggcaggagcaggaggaggggcaggaggggcaggaggggcaggagcaggaggaggggcaggagcaggaggaggggcaggaggggcaggagcaggaggaggggcaggaggggcaggaggggcaggagcaggaggaggggcaggagcaggaggggcaggaggggcaggaggggcaggagcaggaggggcaggagcaggaggaggggcaggaggggcaggaggggcaggagcaggaggggcaggagcaggaggggcaggagcaggaggggcaggagcaggaggggcaggaggggcaggagcaggaggggcaggaggggcaggagcaggaggggcaggaggggcaggagcaggaggaggggcaggaggggcaggagcaggaggaggggcaggaggggcaggagcaggaggggcaggaggggcaggagcaggaggggcaggaggggcaggagcaggaggggcaggaggggcaggagcaggaggaggggcaggagcaggaggggcaggagcaggaggtggaggccggggtcgaggaggcagtggaggccggggtcgaggaggtagtggaggccggggtcgaggaggtagtggaggccgccggggtagaggacgtgaaagagccagggggggaagtcgtgaaagagccagggggagaggtcgtggacgtggagaaaagaggcccaggagtcccagtagtcagtcatcatcatccgggtctccaccgcgcaggccccctccaggtagaaggccatttttccaccctgtaggggaagccgattattttgaataccaccaagaaggtggcccagatggtgagcctgacgtgcccccgggagcgatagagcagggccccgcagatgacccaggagaaggcccaagcactggaccccggggtcagggtgatggaggcaggcgcaaaaaaggagggtggtttggaaagcatcgtggtcaaggaggttccaacccgaaatttgagaacattgcagaaggtttaagagctctcctggctaggagtcacgtagaaaggactaccgacgaaggaacttgggtcgccggtgtgttcgtatatggaggtagtaagacctccctttacaacctaaggcgaggaactgcccttgctattccacaatgtcgtcttacaccattgagtcgtctcccctttggaatggcccctggacccggcccacaacctggcccgctaagggagtccattgtctgttatttcatggtctttttacaaactcatatatttgctgaggttttgaaggatgcgattaaggaccttgttatgacaaagcccgctcctacctgcaatatcagggtgactgtgtgcagctttgacgatggagtagatttgcctccctggtttccacctatggtggaaggggctgccgcggagggtgatgacggagatgacggagatgaaggaggtgatggagatgagggtgaggaagggcaggagtgatgtaacttgttaggagacgccctcaatcgtattaaaagccgtgtattcccccgcactaaagaataaatccccagtagacatcatgcgtgctgttggtgtatttctggccatctgtcttgtcaccattttcgtcctcccaacatggggcaattgggcatacccatgttgtcacgtcactcagctccgcgctcaacaccttctcgcgttggaaaacattagcgacatttacctggtgagcaatcagacatgcgacggctttagcctggcctccttaaattcacctaagaatgggagcaaccagcaggaaaaggacaagcagcgaaaattcacgcccccttgggaggtggcggcatatgcaaaggatagcactcccactctactactgggtatcatatgctgactgtatatgcatgaggatagcatatgctacccggatacagattaggatagcatatactacccagatatagattaggatagcatatgctacccagatatagattaggatagcctatgctacccagatataaattaggatagcatatactacccagatatagattaggatagcatatgctacccagatatagattaggatagcctatgctacccagatatagattaggatagcatatgctacccagatatagattaggatagcatatgctatccagatatttgggtagtatatgctacccagatataaattaggatagcatatactaccctaatctctattaggatagcatatgctacccggatacagattaggatagcatatactacccagatatagattaggatagcatatgctacccagatatagattaggatagcctatgctacccagatataaattaggatagcatatactacccagatatagattaggatagcatatgctacccagatatagattaggatagcctatgctacccagatatagattaggatagcatatgctatccagatatttgggtagtatatgctacccatggcaacattagcccaccgtgctctcagcgacctcgtgaatatgaggaccaacaaccctgtgcttggcgctcaggcgcaagtgtgtgtaatttgtcctccagatcgcagcaatcgcgcccctatcttggcccgcccacctacttatgcaggtattccccggggtgccattagtggttttgtgggcaagtggtttgaccgcagtggttagcggggttacaatcagccaagttattacacccttattttacagtccaaaaccgcagggcggcgtgtgggggctgacgcgatcgctgttccttaggacccttttactaaccctaattcgatagcatatgcttcccgttgggtaacatatgctattgaattagggttagtctggatagtatatactactacccgggaagcatatgctacccgtttagggttaacaagggggccttataaacactattgctaatgccctcttgagggtccgcttatcggtagctacacaggcccctctgattgacgttggtgtagcctcccgtagtcttcctgggcccctgggaggtacatgtcccccagcattggtgtaagagcttcagccaagagttacacataaaggcaatgttgtgttgcagtccacagactgcaaagtctgctccaggatgaaagccactcagtgttggcaaatgtgcacatccatttataaggatgtcaactacagtcagagaacccctttgtgtttggtccccccccgtgtcacatgtggaacagggcccagttggcaagttgtaccaaccaactgaagggattacatgcactgccccgcgaagaaggggcagagatgtcgtagtcaggtttagttcgtccggggcggggatctcgacattgattattgactagttattaatagtaatcaattacggggtcattagttcatagcccatatatggagttccgcgttacataacttacggtaaatggcccgcctggctgaccgcccaacgacccccgcccattgacgtcaataatgacgtatgttcccatagtaacgccaatagggactttccattgacgtcaatgggtggagtatttacggtaaactgcccacttggcagtacatcaagtgtatcatatgccaagtacgccccctattgacgtcaatgacggtaaatggcccgcctggcattatgcccagtacatgaccttatgggactttcctacttggcagtacatctacgtattagtcatcgctattaccatggtcgaggtgagccccacgttctgcttcactctccccatctcccccccctccccacccccaattttgtatttatttattttttaattattttgtgcagcgatgggggcggggggggggggggggcgcgcgccaggcggggcggggcggggcgaggggcggggcggggcgaggcggagaggtgcggcggcagccaatcagagcggcgcgctccgaaagtttccttttatggcgaggcggcggcggcggcggccctataaaaagcgaagcgcgcggcgggcgggagtcgctgcgcgttgccctcgccccgtgccccgctccgccgccgcctcgcgccgcccgccccggctctgactgaccgcgttactcccacaggtgagcgggcgggacggcccttctcctccgggctgtaattagcgcttggtttaatgacggcttgtttcttttctgtggctgcgtgaaagccttgaggggctccgggagggccctttgtgcggggggagcggctcggggggtgcgtgcgtgtgtgtgtgcgtggggagcgccgcgtgcggctccgcgctgcccggcggctgtgagcgctgcgggcgcggcgcggggctttgtgcgctccgcagtgtgcgcgaggggagcgcggccgggggcggtgccccgcggtgcggggggggctgcgaggggaacaaaggctgcgtgcggggtgtgtgcgtgggggggtgagcagggggtgtgggcgcgtcggtcgggctgcaaccccccctgcacccccctccccgagttgctgagcacggcccggcttcgggtgcggggctccgtacggggcgtggcgcggggctcgccgtgccgggcggggggtggcggcaggtgggggtgccgggcggggcggggccgcctcgggccggggagggctcgggggaggggcgcggcggcccccggagcgccggcggctgtcgaggcgcggcgagccgcagccattgccttttatggtaatcgtgcgagagggcgcagggacttcctttgtcccaaatctgtgcggagccgaaatctgggaggcgccgccgcaccccctctagcgggcgcggggcgaagcggtgcggcgccggcaggaaggaaatgggcggggagggccttcgtgcgtcgccgcgccgccgtccccttctccctctccagcctcggggctgtccgcggggggacggctgccttcgggggggacggggcagggcggggttcggcttctggcgtgtgaccggcggctctagagcctctgctaaccatgttcatgccttcttctttttcctacagctcctgggcaacgtgctggttattgtgctgtctcatcattttggcaaagaattaaccctcactaaaggggtaccgggccccccctcgaatgactacgtccggcgttccatttggcatgacactacgaccaacacgatctcggttgtctcggcgcactccgtacagtagggatcgcctacctccttttgagacagagacccgcgctaccatactggaggatcatccgctgctgcccgaatgtaacactttgacaatgcacaacgtgagttacgtgcgaggtcttccctgcagtgtgggatttacgctgattcaggaatgggttgttccctgggatatggttctgacgcgggaggagcttgtaatcctgaggaagtgtatgcacgtgtgcctgtgttgtgccaacattgatatcatgacgagcatgatgatccatggttacgagtcctgggctctccactgtcattgttccagtcccggttccctgcagtgcatagccggcgggcaggttttggccagctggtttaggatggtggtggatggcgccatgtttaatcagaggtttatatggtaccgggaggtggtgaattacaacatgccaaaagaggtaatgtttatgtccagcgtgtttatgaggggtcgccacttaatctacctgcgcttgtggtatgatggccacgtgggttctgtggtccccgccatgagctttggatacagcgccttgcactgtgggattttgaacaatattgtggtgctgtgctgcagttactgtgctgatttaagtgagatcagggtgcgctgctgtgcccggaggacaaggcgtctcatgctgcgggcggtgcgaatcatcgctgaggagaccactgccatgttgtattcctgcaggacggagcggcggcggcagcagtttattcgcgcgctgctgcagcaccaccgccctatcctgatgcacgattatgactctacccccatgggccgcgactctagatcataatcagccataccacatttgtagaggttttacttgctttaaaaaacctcccacacctccccctgaacctgaaacataaaatgaatgcaattgttgttgttaacttgtttattgcagcttataatggttacaaataaagcaatagcatcacaaatttcacaaataaagcatttttttcactgcattctagttgtggtttgtccaaactcatcaatgtatcttaaggcgtaaattgtaagcgttaatattttgttaaaattcgcgttaaatttttgttaaatcagctcattttttaaccaataggccgaaatcggcaaaatcccttataaatcaaaagaatagaccgagatagggttgagtgttgttccagtttggaacaagagtccactattaaagaacgtggactccaacgtcaaagggcgaaaaaccgtctatcagggcgatggcccactacgtgaaccatcaccctaatcaagttttttggggtcgaggtgccgtaaagcactaaatcggaaccctaaagggagcccccgatttagagcttgacggggaaagccggcgaacgtggcgagaaaggaagggaagaaagcgaaaggagcgggcgctagggcgctggcaagtgtagcggtcacgctgcgcgtaaccaccacacccgccgcgcttaatgcgccgctacagggcgcgtcaggtggcacttttcggggaaatgtgcgcggaacccctatttgtttatttttctaaatacattcaaatatgtatccgctcatgagacaataaccctgataaatgcttcaataatattgaaaaaggaagagtcctgaggcggaaagaaccagctgtggaatgtgtgtcagttagggtgtggaaagtccccaggctccccagcaggcagaagtatgcaaagcatgcatctcaattagtcagcaaccaggtgtggaaagtccccaggctccccagcaggcagaagtatgcaaagcatgcatctcaattagtcagcaaccatagtcccgcccctaactccgcccatcccgcccctaactccgcccagttccgcccattctccgccccatggctgactaattttttttatttatgcagaggccgaggccgcctcggcctctgagctattccagaagtagtgaggaggcttttttggaggcctaggcttttgcaaagatcatcaagagacaggatgaggatcgtttcgcatgattgaacaagatggattgcacgcaggttctccggccgcttgggtggagaggctattcggctatgactgggcacaacagacaatcggctgctctgatgccgccgtgttccggctgtcagcgcaggggcgcccggttctttttgtcaagaccgacctgtccggtgccctgaatgaactgcaagacgaggcagcgcggctatcgtggctggccacgacgggcgttccttgcgcagctgtgctcgacgttgtcactgaagcgggaagggactggctgctattgggcgaagtgccggggcaggatctcctgtcatctcaccttgctcctgccgagaaagtatccatcatggctgatgcaatgcggcggctgcatacgcttgatccggctacctgcccattcgaccaccaagcgaaacatcgcatcgagcgagcacgtactcggatggaagccggtcttgtcgatcaggatgatctggacgaagagcatcaggggctcgcgccagccgaactgttcgccaggctcaaggcgagcatgcccgacggcgaggatctcgtcgtgacccatggcgatgcctgcttgccgaatatcatggtggaaaatggccgcttttctggattcatcgactgtggccggctgggtgtggcggaccgctatcaggacatagcgttggctacccgtgatattgctgaagagcttggcggcgaatgggctgaccgcttcctcgtgctttacggtatcgccgctcccgattcgcagcgcatcgccttctatcgccttcttgacgagttcttctgagcgggactctggggttcgaaatgaccgaccaagcgacgcccaacctgccatcacgagatttcgattccaccgccgccttctatgaaaggttgggcttcggaatcgttttccgggacgccggctggatgatcctccagcgcggggatctcatgctggagttcttcgcccaccctagggggaggctaactgaaacacggaaggagacaataccggaaggaacccgcgctatgacggcaataaaaagacagaataaaacgcacggtgttgggtcgtttgttcataaacgcggggttcggtcccagggctggcactctgtcgataccccaccgagaccccattggggccaatacgcccgcgtttcttccttttccccaccccaccccccaagttcgggtgaaggcccagggctcgcagccaacgtcggggcggcaggccctgccatagcctcaggttactcatatatactttagattgatttaaaacttcatttttaatttaaaaggatctaggtgaagatcctttttgataatctcatgaccaaaatcccttaacgtgagttttcgttccactgagcgtcagaccccgtagaaaagatcaaaggatcttc

SEQ ID NO: 7 - DNA, 3998 bp, synthetic construct
  misc_feature 1..3998: note = plasmid
  source 1..3998: mol_type = other DNA
tcgcgcgtttcggtgatgacggtgaaaacctctgacacatgcagctcccggagactgtcacagcttgtctgtaagcggatgccgggagcagacaagcccgtcagggcgcgtcagcgggtgttggcgggtgtcggggctggcttaactatgcggcatcagagcagattgtactgagagtgcaccatatgcggtgtgaaataccgcacagatgcgtaaggagaaaataccgcatcaggcgccattcgccattcaggctgcgcaactgttgggaagggcgatcggtgcgggcctcttcgctattacgccagctggcgaaagggggatgtgctgcaaggcgattaagttgggtaacgccagggttttcccagtcacgacgttgtaaaacgacggccagtgaattgacgcgtattgggatgtgatgcggttttggcagtacatcaatgggcgtggatagcggtttgactcacggggatttccaagtctccaccccattgacgtcaatgggagtttgttttggaaccaaaatcaacgggactttccaaaatgtcgtaacaactccgccccattgacgcaaatgggcggtaggcgtgtacggtgggaggtctatataagcagagctctccctatcagtgatagagatctccctatcagtgatagagatcgtcgacgagctcgtttagtgaaccgtcagatcgcctggagacgccatccacgctgttttgacctccatagaagacaccgggaccgatccagcctccggactctagcgtttaaacttaagcttgccaccatgactacgtccggcgttccatttggcatgacactacgaccaacacgatctcggttgtctcggcgcactccgtacagtagggatcgcctacctccttttgagacagagacccgcgctaccatactggaggatcatccgctgctgcccgaatgtaacactttgacaatgcacaacgtgagttacgtgcgaggtcttccctgcagtgtgggatttacgctgattcaggaatgggttgttccctgggatatggttctgacgcgggaggagcttgtaatcctgaggaagtgtatgcacgtgtgcctgtgttgtgccaacattgatatcatgacgagcatgatgatccatggttacgagtcctgggctctccactgtcattgttccagtcccggttccctgcagtgcatagccggcgggcaggttttggccagctggtttaggatggtggtggatggcgccatgtttaatcagaggtttatatggtaccgggaggtggtgaattacaacatgccaaaagaggtaatgtttatgtccagcgtgtttatgaggggtcgccacttaatctacctgcgcttgtggtatgatggccacgtgggttctgtggtccccgccatgagctttggatacagcgccttgcactgtgggattttgaacaatattgtggtgctgtgctgcagttactgtgctgatttaagtgagatcagggtgcgctgctgtgcccggaggacaaggcgtctcatgctgcgggcggtgcgaatcatcgctgaggagaccactgccatgttgtattcctgcaggacggagcggcggcggcagcagtttattcgcgcgctgctgcagcaccaccgccctatcctgatgcacgattatgactctacccccatgtaggcggccgctcgagtctagagggcccgtttaaacccgctgatcagcctcgatgcggtgggctctatggatcccaatggcgcgccgagcttggcgtaatcatggtcatagctgtttcctgtgtgaaattgttatccgctcacaattccacacaacatacgagccggaagcataaagtgtaaagcctggggtgcctaatgagtgagctaactcacattaattgcgttgcgctcactgcccgctttccagtcgggaaacctgtcgtgccagctgcattaatgaatcggccaacgcgcggggagaggcggtttgcgtattgggcgctgttccgcttcctcgctcactgactcgctgcgctcggtcgttcggctgcggcgagcggtatcagctcactcaaaggcggtaatacggttatccacagaatcaggggataacgcaggaaagaacatgtgagcaaaaggccagcaaaaggccaggaaccgtaaaaaggccgcgttgctggcgtttttccataggctccgcccccctgacgagcatcacaaaaatcgacgctcaagtcagaggtggcgaaacccgacaggactataaagataccaggcgtttccccctggaagctccctcgtgcgctctcctgttccgaccctgccgcttaccggatacctgtccgcctttctcccttcgggaagcgtggcgctttctcatagctcacgctgtaggtatctcagttcggtgtaggtcgttcgctccaagctgggctgtgtgcacgaaccccccgttcagcccgaccgctgcgccttatccggtaactatcgtcttgagtccaacccggtaagacacgacttatcgccactggcagcagccactggtaacaggattagcagagcgaggtatgtaggcggtgctacagagttcttgaagtggtggcctaactacggctacactagaagaacagtatttggtatctgcgctctgctgaagccagttaccttcggaaaaagagttggtagctcttgatccggcaaacaaaccaccgctggtagcggtggtttttttgtttgcaagcagcagattacgcgcagaaaaaaaggatctcaagaagatcctttgatcttttctacggggtctgacgctcagtggaacgaaaactcacgttaagggattttggtcatgagattatcaaaaaggatcttcacctagatccttttaaattaaaaatgaagttttaaatcaatctaaagtatatatgagtaaacttggtctgacagttaccaatgcttaatcagtgaggcacctatctcagcgatctgtctatttcgttcatccatagttgcctgactccccgtcgtgtagataactacgatacgggagggcttaccatctggccccagtgctgcaatgataccgcgagaaccacgctcaccggctccagatttatcagcaataaaccagccagccggaagggccgagcgcagaagtggtcctgcaactttatccgcctccatccagtctattaattgttgccgggaagctagagtaagtagttcgccagttaatagtttgcgcaacgttgttgccattgctacaggcatcgtggtgtcacgctcgtcgtttggtatggcttcattcagctccggttcccaacgatcaaggcgagttacatgatcccccatgttgtgcaaaaaagcggttagctccttcggtcctccgatcgttgtcagaagtaagttggccgcagtgttatcactcatggttatggcagcactgcataattctcttactgtcatgccatccgtaagatgcttttctgtgactggtgagtactcaaccaagtcattctgagaatagtgtatgcggcgaccgagttgctcttgcccggcgtcaatacgggataataccgcgccacatagcagaactttaaaagtgctcatcattggaaaacgttcttcggggcgaaaactctcaaggatcttaccgctgttgagatccagttcgatgtaacccactcgtgcacccaactgatcttcagcatcttttactttcaccagcgtttctgggtgagcaaaaacaggaaggcaaaatgccgcaaaaaagggaataagggcgacacggaaatgttgaatactcatactcttcctttttcaatattattgaagcatttatcagggttattgtctcatgagcggatacatatttgaatgtatttagaaaaataaacaaataggggttccgcgcacatttccccgaaaagtgccacctgacgtctaagaaaccattattatcatgacattaacctataaaaataggcgtatcacgaggcccttttgtc

SEQ ID NO: 8 - DNA, 22 bp, synthetic construct
  misc_feature 1..22: note = primer
  source 1..22: mol_type = other DNA
tggtttaggatggtggtggatg

SEQ ID NO: 9 - DNA, 21 bp, synthetic construct
  misc_feature 1..21: note = primer
  source 1..21: mol_type = other DNA
cgcaggtagattaagtggcga

SEQ ID NO: 10 - DNA, 24 bp, synthetic construct
  misc_feature 1..24: note = priobe
  source 1..24: mol_type = other DNA
gaggtaatgtttatgtccagcgtg

SEQ ID NO: 11 - DNA, 21 bp, synthetic construct
  misc_feature 1..21: note = primer
  source 1..21: mol_type = other DNA
ggaacccctagtgatggagtt

SEQ ID NO: 12 - DNA, 16 bp, synthetic construct
  misc_feature 1..16: note = primer
  source 1..16: mol_type = other DNA
cggcctcagtgagcga

SEQ ID NO: 13 - DNA, 21 bp, synthetic construct
  misc_feature 1..21: note = probe
  source 1..21: mol_type = other DNA
cactccctctctgcgcgctcg

SEQ ID NO: 14 - DNA, 9266 bp, synthetic construct
  misc_feature 1..9266: note = plasmid
  source 1..9266: mol_type = other DNA
aaattgtaagcgttaatattttgttaaaattcgcgttaaatttttgttaaatcagctcattttttaaccaataggccgaaatcggcaaaatcccttataaatcaaaagaatagaccgagatagggttgagtgttgttccagtttggaacaagagtccactattaaagaacgtggactccaacgtcaaagggcgaaaaaccgtctatcagggcgatggcccactacgtgaaccatcaccctaatcaagttttttggggtcgaggtgccgtaaagcactaaatcggaaccctaaagggagcccccgatttagagcttgacggggaaagccggcgaacgtggcgagaaaggaagggaagaaagcgaaaggagcgggcgctagggcgctggcaagtgtagcggtcacgctgcgcgtaaccaccacacccgccgcgcttaatgcgccgctacagggcgcgatggatccgcggccgcttaagccataccaatggtttactccctatcagtgatagagaacgtatgaagagtttactccctatcagtgatagagaacgtatgcagactttactccctatcagtgatagagaacgtataaggagtttactccctatcagtgatagagaacgtatgaccagtttactccctatcagtgatagagaacgtatctacagtttactccctatcagtgatagagaacgtatatccagtttactccctatcagtgatagagaacgtatgtcgaggtaggcgtgtacggtgggcgcctataaaagcagagctcgtttagtgaaccgtcagatcgcctggagcaattccacaacacttttgtcttatacttggtttagtgaaccgtcagatcagatctttgtcgatcctaccatccactcgacacacccgccagcggccgatggcccttagtaagcacggcctgactaaggacatgaccatgaagtaccatatggagggctcggtggacgggcacaagttcgtgattacgggccacgggaacggcaacccattcgaggggaaacagacaatgaacctgtgtgtggtggaaggcggacccctgcccttctcggaggacatcctgtccgcaacctttgactacggcaatcgcgtgttcacagagtatccacagggtatggtggatttctttaagaacagctgtcccgcaggatacacctggcaccgcagcctgctcttcgaggacggggcggtgtgtaccacctccgctgatatcaccgtgtccgtcgaggagaactgcttctaccacaacagcaaattccacggcgtgaactttcctgccgacgggcctgtgatgaagaaaatgactacgaattgggagcccagctgcgagaaaatcatcccggtccctcgtcagggaatcttgaagggcgacatcgcaatgtacctcctgctcaaggacgggggaagataccgatgccagttcgataccatctacaaggcaaagtccgatcccaaggagatgccagagtggcacttcatccagcacaaactcacccgcgaggaccgctcagatgccaagaaccagaagtggcaactggtcgagcacgccgtggcatcccgtagcgccctgccagggtaatcgttactggccgaagccgcttggaataaggccggtgtgcgtttgtctatatgttattttccaccatattgccgtcttttggcaatgtgagggcccggaaacctggccctgtcttcttgacgagcattcctaggggtctttcccctctcgccaaaggaatgcaaggtctgttgaatgtcgtgaaggaagcagttcctctggaagcttcttgaagacaaacaacgtctgtagcgaccctttgcaggcagcggaaccccccacctggcgacaggtgcctctgcggccaaaagccacgtgtataagatacacctgcaaaggcggcacaaccccagtgccacgttgtgagttggatagttgtggaaagagtcaaatggctcccctcaagcgtattcaacaaggggctgaaggatgcccagaaggtaccccattgtatgggatctgatctggggcctcggtgcacatgctttacatgtgtttagtcgaggttaaaaaacgtctaggccccccgaaccacggggacgtggttttctttgaaaaacacgatgataatacatgactacgtccggcgttccatttggcatgacactacgaccaacacgatctcggttgtctcggcgcactccgtacagtagggatcgcctacctccttttgagacagagacccgcgctaccatactggaggatcatccgctgctgcccgaatgtaacactttgacaatgcacaacgtgagttacgtgcgaggtcttccctgcagtgtgggatttacgctgattcaggaatgggttgttccctgggatatggttctgacgcgggaggagcttgtaatcctgaggaagtgtatgcacgtgtgcctgtgttgtgccaacattgatatcatgacgagcatgatgatccatggttacgagtcctgggctctccactgtcattgttccagtcccggttccctgcagtgcatagccggcgggcaggttttggccagctggtttaggatggtggtggatggcgccatgtttaatcagaggtttatatggtaccgggaggtggtgaattacaacatgccaaaagaggtaatgtttatgtccagcgtgtttatgaggggtcgccacttaatctacctgcgcttgtggtatgatggccacgtgggttctgtggtccccgccatgagctttggatacagcgccttgcactgtgggattttgaacaatattgtggtgctgtgctgcagttactgtgctgatttaagtgagatcagggtgcgctgctgtgcccggaggacaaggcgtctcatgctgcgggcggtgcgaatcatcgctgaggagaccactgccatgttgtattcctgcaggacggagcggcggcggcagcagtttattcgcgcgctgctgcagcaccaccgccctatcctgatgcacgattatgactctacccccatgtaggcggccgctcgagtctagagggcccgtttaaacccgctgatcagcctcgactgtgccttctagttgccagccatctgttgtttgcccctcccccgtgccttccttgaccctggaaggtgccactcccactgtcctttcctaataaaatgaggaaattgcatcgcattgtctgagtaggtgtcattctattctggggggtggggtggggcaggacagcaagggggaggattgggaagacaatagcaggcatgctggggatgcggtgggctctatggtcatgttctagactgtaagcggccgctacgtcgacgtttaaaccatacaatcagcattggtagctgctgtattgctacttgtgattgctccatgtttttctaggtctcgactgcagaattaattccaggcggggaggcggcccaaagggagatccgactcgtctgagggcgaaggcgaagacgcggaagaggccgcagagccggcagcaggccgcgggaaggaaggtccgctggattgagggccgaagggacgtagcagaaggacgtcccgcgcagaatccaggtggcaacacaggcgagcagccatggaaaggacgtcagcttccccgacaacaccacggaattgtcagtgcccaacagccgagcccctgtccagcagcgggcaaggcaggcggcgatgagttccgccgtggcaatagggagggggaaagcgaaagtcccggaaaggagctgacaggtggtggcaatgccccaaccagtgggggttgcgtcagcaaacacagtgcacaccacgccacgttgcctgacaacgggccacaactcctcataaagagacagcaaccaggatttatacaaggaggagaaaatgaaagccatacgggaagcaatagcatgatacaaaggcattaaagcagcgtatccacatagcgtaaaaggagcaacatagttaagaataccagtcaatctttcacaaattttgtaatccagaggttgattgttccagacgcgttcagaagaactcgtcaagaaggcgatagaaggcgatgcgctgcgaatcgggagcggcgataccgtaaagcacgaggaagcggtcagcccattcgccgccaagctcttcagcaatatcacgggtagccaacgctatgtcctgatagcggtccgccacacccagccggccacagtcgatgaatccagaaaagcggccattttccaccatgatattcggcaagcaggcatcgccatgggtcacgacgagatcctcgccgtcgggcatgcgcgccttgagcctggcgaacagttcggctggcgcgagcccctgatgctcttcgtccagatcatcctgatcgacaagaccggcttccatccgagtacgtgctcgctcgatgcgatgtttcgcttggtggtcgaatgggcaggtagccggatcaagcgtatgcagccgccgcattgcatcagccatgatggatactttctcggcaggagcaaggtgagatgacaggagatcctgccccggcacttcgcccaatagcagccagtcccttcccgcttcagtgacaacgtcgagcacagctgcgcaaggaacgcccgtcgtggccagccacgatagccgcgctgcctcgtcctgcagttcattcagggcaccggacaggtcggtcttgacaaaaagaaccgggcgcccctgcgctgacagccggaacacggcggcatcagagcagccgattgtctgttgtgcccagtcatagccgaatagcctctccacccaagcggccggagaacctgcgtgcaatccatcttgttcagccatggcggcgttaactgcaggtcgaaaggcccggagatgaggaagaggagaacagcgcggcagacgtgcgcttttgaagcgtgcagaatgccgggcctccggaggaccttcgggcgcccgccccgcccctgagcccgcccctgagcccgcccccggacccaccccttcccagcctctgagcccagaaagcgaaggagcaaagctgctattggccgctgccccaaaggcctacccgcttccattgctcagcggtgctgtccatctgcacgagactagtgagacgtgctacttccatttgtcacgtcctgcacgacgcgagctgcggggcgggggggaacttcctgactaggggaggagtagaaggtggcgcgaaggggccaccaaagaacggagccggttggcgcctaccggtggatgtggaatgtgtgcgaggccagaggccacttgtgtagcgccaagtgcccagcggggctgctaaagcgcatgctccagactgccttgggaaaagcgcctcccctacccggtagaattggatctagttacccggggagcatgtcaaggtcaaaatcgtcaagagcgtcagcaggcagcatatcaaggtcaaagtcgtcaagggcatcggctgggagcatgtctaagtcaaaatcgtcaagggcgtcggtcggcccgccgctttcgcactttagctgtttctccaggccacatatgattagttccaggccgaaaaggaaggcaggttcggctccctgccggtcgaacagctcaattgcttgtttcagaagtgggggcatagaatcggtggtaggtgtctctctttcctcttttgctacttgatgctcctgttcctccaatacgcagcccagtgtaaagtggcccacggcggacagagcgtacagtgcgttctccagggagaagccttgctgacacaggaacgcgagctgattttccagggtttcgtactgtttctctgttgggcgggtgccgagatgcactttagccccgtcgcgatgtgagaggagagcacagcggtatgacttggcgttgttccgcagaaagtcttgccatgactcgccttccagggggcaggagtgggtatgatgcctgtccagcatctcgattggcagggcatcgagcagggcccgcttgttcttcacgtgccagtacagggtaggctgctcaactcccagcttttgagcgagtttccttgtcgtcaggccttcgataccgactccattgagtaattccagagcagagtttatgactttgctcttgtccagtctagacatggtgaactagaatttaaatcctgcaggttcacgacacctgaaatggaagaaaaaaactttgaaccactgtctgaggcttgagaatgaaccaagatccaaactcaaaaagggcaaattccaaggagaattacatcaagtgccaagctggcctaacttcagtctccacccactcagtgtggggaaactccatcgcataaaacccctccccccaacctaaagacgacgtactccaaaagctcgagaactaatcgaggtgcctggacggcgcccggtactccgtggagtcacatgaagcgacggctgaggacggaaaggcccttttcctttgtgtgggtgactcacccgcccgctctcccgagcgccgcgtcctccattttgagctccctgcagcagggccgggaagcggccatctttccgctcacgcaactggtgccgaccgggccagccttgccgcccagggcggggcgatacacggcggcgcgaggccaggcaccagagcaggccggccagcttgagactacccccgtccgattctcggtggccgcgctcgcaggccccgcctcgccgaacatgtgcgctgggacgcacgggccccgtcgccgcccgcggccccaaaaaccgaaataccagtgtgcagatcttggcccgcatttacaagactatcttgccagaaaaaaagcgtcgcagcaggtcatcaaaaattttaaatggctagagacttatcgaaagcagcgagacaggcgcgaaggtgccaccagattcgcacgcggcggccccagcgcccaagccaggcctcaactcaagcacgaggcgaaggggctccttaagcgcaaggcctcgaactctcccacccacttccaacccgaagctcgggatcaagaatcacgtactgcagccaggggcgtggaagtaattcaaggcacgcaagggccataacccgtaaagaggccaggcccgcgggaaccacacacggcacttacctgtgttctggcggcaaacccgttgcgaaaaagaacgttcacggcgactactgcacttatatacggttctcccccaccctcgggaaaaaggcggagccagtacacgacatcactttcccagtttaccccgcgccaccttctctaggcaccggttcaattgccgacccctccccccaacttctcggggactgtgggcgatgtgcgctctgcccactgacgggcaccggagcctcacgaattcgatatcgataaactggatctctgctgtccctgtaataaacccgaatatgatcagctcactcaaaggcggtaatacggttatccacagaatcaggggataacgcaggaaagaacatgtgagcaaaaggccagcaaaaggccaggaaccgtaaaaaggccgcgttgctggcgtttttccataggctccgcccccctgacgagcatcacaaaaatcgacgctcaagtcagaggtggcgaaacccgacaggactataaagataccaggcgtttccccctggaagctccctcgtgcgctctcctgttccgaccctgccgcttaccggatacctgtccgcctttctcccttcgggaagcgtggcgctttctcatagctcacgctgtaggtatctcagttcggtgtaggtcgttcgctccaagctgggctgtgtgcacgaaccccccgttcagcccgaccgctgcgccttatccggtaactatcgtcttgagtccaacccggtaagacacgacttatcgccactggcagcagccactggtaacaggattagcagagcgaggtatgtaggcggtgctacagagttcttgaagtggtggcctaactacggctacactagaagaacagtatttggtatctgcgctctgctgaagccagttaccttcggaaaaagagttggtagctcttgatccggcaaacaaaccaccgctggtagcggtggtttttttgtttgcaagcagcagattacgcgcagaaaaaaaggatctcaagaagatcctttgatcttttctacggggtctgacgctcagtggaacgaaaactcacgttaagggattttggtcatgagattatcaaaaaggatcttcacctagatccttttaaattaaaaatgaagttttaaatcaatctaaagtatatatgagtaaacttggtctgacagttaccaatgcttaatcagtgaggcacctatctcagcgatctgtctatttcgttcatccatagttgcctgactccccgtcgtgtagataactacgatacgggagggcttaccatctggccccagtgctgcaatgataccgcgagacccacgctcaccggctccagatttatcagcaataaaccagccagccggaagggccgagcgcagaagtggtcctgcaactttatccgcctccatccagtctattaattgttgccgggaagctagagtaagtagttcgccagttaatagtttgcgcaacgttgttgccattgctacaggcatcgtggtgtcacgctcgtcgtttggtatggcttcattcagctccggttcccaacgatcaaggcgagttacatgatcccccatgttgtgcaaaaaagcggttagctccttcggtcctccgatcgttgtcagaagtaagttggccgcagtgttatcactcatggttatggcagcactgcataattctcttactgtcatgccatccgtaagatgcttttctgtgactggtgagtactcaaccaagtcattctgagaatagtgtatgcggcgaccgagttgctcttgcccggcgtcaatacgggataataccgcgccacatagcagaactttaaaagtgctcatcattggaaaacgttcttcggggcgaaaactctcaaggatcttaccgctgttgagatccagttcgatgtaacccactcgtgcacccaactgatcttcagcatcttttactttcaccagcgtttctgggtgagcaaaaacaggaaggcaaaatgccgcaaaaaagggaataagggcgacacggaaatgttgaatactcatactcttcctttttcaatattattgaagcatttatcagggttattgtctcatgagcggatacatatttgaatgtatttagaaaaataaacaaataggggttccgcgcacatttccccgaaaagtgccacct

SEQ ID NO: 15 - DNA, 8985 bp, synthetic construct
  misc_feature 1..8985: note = plasmid
  source 1..8985: mol_type = other DNA
aaattgtaagcgttaatattttgttaaaattcgcgttaaatttttgttaaatcagctcattttttaaccaataggccgaaatcggcaaaatcccttataaatcaaaagaatagaccgagatagggttgagtgttgttccagtttggaacaagagtccactattaaagaacgtggactccaacgtcaaagggcgaaaaaccgtctatcagggcgatggcccactacgtgaaccatcaccctaatcaagttttttggggtcgaggtgccgtaaagcactaaatcggaaccctaaagggagcccccgatttagagcttgacggggaaagccggcgaacgtggcgagaaaggaagggaagaaagcgaaaggagcgggcgctagggcgctggcaagtgtagcggtcacgctgcgcgtaaccaccacacccgccgcgcttaatgcgccgctacagggcgcgatggatccgcggccgcttaagccataccaatggtttactccctatcagtgatagagaacgtatgaagagtttactccctatcagtgatagagaacgtatgcagactttactccctatcagtgatagagaacgtataaggagtttactccctatcagtgatagagaacgtatgaccagtttactccctatcagtgatagagaacgtatctacagtttactccctatcagtgatagagaacgtatatccagtttactccctatcagtgatagagaacgtatgtcgaggtaggcgtgtacggtgggcgcctataaaagcagagctcgtttagtgaaccgtcagatcgcctggagcaattccacaacacttttgtcttatacttggtttagtgaaccgtcagatcagatctttgtcgatcctaccatccactcgacacacccgccagcggccgatggcccttagtaagcacggcctgactaaggacatgaccatgaagtaccatatggagggctcggtggacgggcacaagttcgtgattacgggccacgggaacggcaacccattcgaggggaaacagacaatgaacctgtgtgtggtggaaggcggacccctgcccttctcggaggacatcctgtccgcaacctttgactacggcaatcgcgtgttcacagagtatccacagggtatggtggatttctttaagaacagctgtcccgcaggatacacctggcaccgcagcctgctcttcgaggacggggcggtgtgtaccacctccgctgatatcaccgtgtccgtcgaggagaactgcttctaccacaacagcaaattccacggcgtgaactttcctgccgacgggcctgtgatgaagaaaatgactacgaattgggagcccagctgcgagaaaatcatcccggtccctcgtcagggaatcttgaagggcgacatcgcaatgtacctcctgctcaaggacgggggaagataccgatgccagttcgataccatctacaaggcaaagtccgatcccaaggagatgccagagtggcacttcatccagcacaaactcacccgcgaggaccgctcagatgccaagaaccagaagtggcaactggtcgagcacgccgtggcatcccgtagcgccctgccagggtaatcgttactggccgaagccgcttggaataaggccggtgtgcgtttgtctatatgttattttccaccatattgccgtcttttggcaatgtgagggcccggaaacctggccctgtcttcttgacgagcattcctaggggtctttcccctctcgccaaaggaatgcaaggtctgttgaatgtcgtgaaggaagcagttcctctggaagcttcttgaagacaaacaacgtctgtagcgaccctttgcaggcagcggaaccccccacctggcgacaggtgcctctgcggccaaaagccacgtgtataagatacacctgcaaaggcggcacaaccccagtgccacgttgtgagttggatagttgtggaaagagtcaaatggctcccctcaagcgtattcaacaaggggctgaaggatgcccagaaggtaccccattgtatgggatctgatctggggcctcggtgcacatgctttacatgtgtttagtcgaggttaaaaaacgtctaggccccccgaaccacggggacgtggttttctttgaaaaacacgatgataatacatgactacgtccggcgttccatttggcatgacactacgaccaacacgatctcggttgtctcggcgcactccgtacagtagggatcgcctacctccttttgagacagagacccgcgctaccatactggaggatcatccgctgctgcccgaatgtaacactttgacaatgcacaacgtgagttacgtgcgaggtcttccctgcagtgtgggatttacgctgattcaggaatgggttgttccctgggatatggttctgacgcgggaggagcttgtaatcctgaggaagtgtatgcacgtgtgcctgtgttgtgccaacattgatatcatgacgagcatgatgatccatggttacgagtcctgggctctccactgtcattgttccagtcccggttccctgcagtgcatagccggcgggcaggttttggccagctggtttaggatggtggtggatggcgccatgtttaatcagaggtttatatggtaccgggaggtggtgaattacaacatgccaaaagaggtaatgtttatgtccagcgtgtttatgaggggtcgccacttaatctacctgcgcttgtggtatgatggccacgtgggttctgtggtccccgccatgagctttggatacagcgccttgcactgtgggattttgaacaatattgtggtgctgtgctgcagttactgtgctgatttaagtgagatcagggtgcgctgctgtgcccggaggacaaggcgtctcatgctgcgggcggtgcgaatcatcgctgaggagaccactgccatgttgtattcctgcaggacggagcggcggcggcagcagtttattcgcgcgctgctgcagcaccaccgccctatcctgatgcacgattatgactctacccccatgtagtcatgtctgtaagcggccgctacgtcgacgtttaaaccatacaatcagcattggtagctgctgtattgctacttgtgattgctccatgtttttctaggtctcgactgcagaattaattccaggcggggaggcggcccaaagggagatccgactcgtctgagggcgaaggcgaagacgcggaagaggccgcagagccggcagcaggccgcgggaaggaaggtccgctggattgagggccgaagggacgtagcagaaggacgtcccgcgcagaatccaggtggcaacacaggcgagcagccatggaaaggacgtcagcttccccgacaacaccacggaattgtcagtgcccaacagccgagcccctgtccagcagcgggcaaggcaggcggcgatgagttccgccgtggcaatagggagggggaaagcgaaagtcccggaaaggagctgacaggtggtggcaatgccccaaccagtgggggttgcgtcagcaaacacagtgcacaccacgccacgttgcctgacaacgggccacaactcctcataaagagacagcaaccaggatttatacaaggaggagaaaatgaaagccatacgggaagcaatagcatgatacaaaggcattaaagcagcgtatccacatagcgtaaaaggagcaacatagttaagaataccagtcaatctttcacaaattttgtaatccagaggttgattgttccagacgcgttcagaagaactcgtcaagaaggcgatagaaggcgatgcgctgcgaatcgggagcggcgataccgtaaagcacgaggaagcggtcagcccattcgccgccaagctcttcagcaatatcacgggtagccaacgctatgtcctgatagcggtccgccacacccagccggccacagtcgatgaatccagaaaagcggccattttccaccatgatattcggcaagcaggcatcgccatgggtcacgacgagatcctcgccgtcgggcatgcgcgccttgagcctggcgaacagttcggctggcgcgagcccctgatgctcttcgtccagatcatcctgatcgacaagaccggcttccatccgagtacgtgctcgctcgatgcgatgtttcgcttggtggtcgaatgggcaggtagccggatcaagcgtatgcagccgccgcattgcatcagccatgatggatactttctcggcaggagcaaggtgagatgacaggagatcctgccccggcacttcgcccaatagcagccagtcccttcccgcttcagtgacaacgtcgagcacagctgcgcaaggaacgcccgtcgtggccagccacgatagccgcgctgcctcgtcctgcagttcattcagggcaccggacaggtcggtcttgacaaaaagaaccgggcgcccctgcgctgacagccggaacacggcggcatcagagcagccgattgtctgttgtgcccagtcatagccgaatagcctctccacccaagcggccggagaacctgcgtgcaatccatcttgttcagccatggcggcgttaactgcaggtcgaaaggcccggagatgaggaagaggagaacagcgcggcagacgtgcgcttttgaagcgtgcagaatgccgggcctccggaggaccttcgggcgcccgccccgcccctgagcccgcccctgagcccgcccccggacccaccccttcccagcctctgagcccagaaagcgaaggagcaaagctgctattggccgctgccccaaaggcctacccgcttccattgctcagcggtgctgtccatctgcacgagactagtgagacgtgctacttccatttgtcacgtcctgcacgacgcgagctgcggggcgggggggaacttcctgactaggggaggagtagaaggtggcgcgaaggggccaccaaagaacggagccggttggcgcctaccggtggatgtggaatgtgtgcgaggccagaggccacttgtgtagcgccaagtgcccagcggggctgctaaagcgcatgctccagactgccttgggaaaagcgcctcccctacccggtagaattggatctagttacccggggagcatgtcaaggtcaaaatcgtcaagagcgtcagcaggcagcatatcaaggtcaaagtcgtcaagggcatcggctgggagcatgtctaagtcaaaatcgtcaagggcgtcggtcggcccgccgctttcgcactttagctgtttctccaggccacatatgattagttccaggccgaaaaggaaggcaggttcggctccctgccggtcgaacagctcaattgcttgtttcagaagtgggggcatagaatcggtggtaggtgtctctctttcctcttttgctacttgatgctcctgttcctccaatacgcagcccagtgtaaagtggcccacggcggacagagcgtacagtgcgttctccagggagaagccttgctgacacaggaacgcgagctgattttccagggtttcgtactgtttctctgttgggcgggtgccgagatgcactttagccccgtcgcgatgtgagaggagagcacagcggtatgacttggcgttgttccgcagaaagtcttgccatgactcgccttccagggggcaggagtgggtatgatgcctgtccagcatctcgattggcagggcatcgagcagggcccgcttgttcttcacgtgccagtacagggtaggctgctcaactcccagcttttgagcgagtttccttgtcgtcaggccttcgataccgactccattgagtaattccagagcagagtttatgactttgctcttgtccagtctagacatggtgaactagaatttaaatcctgcaggttcacgacacctgaaatggaagaaaaaaactttgaaccactgtctgaggcttgagaatgaaccaagatccaaactcaaaaagggcaaattccaaggagaattacatcaagtgccaagctggcctaacttcagtctccacccactcagtgtggggaaactccatcgcataaaacccctccccccaacctaaagacgacgtactccaaaagctcgagaactaatcgaggtgcctggacggcgcccggtactccgtggagtcacatgaagcgacggctgaggacggaaaggcccttttcctttgtgtgggtgactcacccgcccgctctcccgagcgccgcgtcctccattttgagctccctgcagcagggccgggaagcggccatctttccgctcacgcaactggtgccgaccgggccagccttgccgcccagggcggggcgatacacggcggcgcgaggccaggcaccagagcaggccggccagcttgagactacccccgtccgattctcggtggccgcgctcgcaggccccgcctcgccgaacatgtgcgctgggacgcacgggccccgtcgccgcccgcggccccaaaaaccgaaataccagtgtgcagatcttggcccgcatttacaagactatcttgccagaaaaaaagcgtcgcagcaggtcatcaaaaattttaaatggctagagacttatcgaaagcagcgagacaggcgcgaaggtgccaccagattcgcacgcggcggccccagcgcccaagccaggcctcaactcaagcacgaggcgaaggggctccttaagcgcaaggcctcgaactctcccacccacttccaacccgaagctcgggatcaagaatcacgtactgcagccaggggcgtggaagtaattcaaggcacgcaagggccataacccgtaaagaggccaggcccgcgggaaccacacacggcacttacctgtgttctggcggcaaacccgttgcgaaaaagaacgttcacggcgactactgcacttatatacggttctcccccaccctcgggaaaaaggcggagccagtacacgacatcactttcccagtttaccccgcgccaccttctctaggcaccggttcaattgccgacccctccccccaacttctcggggactgtgggcgatgtgcgctctgcccactgacgggcaccggagcctcacgaattcgatatcgataaactggatctctgctgtccctgtaataaacccgaatatgatcagctcactcaaaggcggtaatacggttatccacagaatcaggggataacgcaggaaagaacatgtgagcaaaaggccagcaaaaggccaggaaccgtaaaaaggccgcgttgctggcgtttttccataggctccgcccccctgacgagcatcacaaaaatcgacgctcaagtcagaggtggcgaaacccgacaggactataaagataccaggcgtttccccctggaagctccctcgtgcgctctcctgttccgaccctgccgcttaccggatacctgtccgcctttctcccttcgggaagcgtggcgctttctcatagctcacgctgtaggtatctcagttcggtgtaggtcgttcgctccaagctgggctgtgtgcacgaaccccccgttcagcccgaccgctgcgccttatccggtaactatcgtcttgagtccaacccggtaagacacgacttatcgccactggcagcagccactggtaacaggattagcagagcgaggtatgtaggcggtgctacagagttcttgaagtggtggcctaactacggctacactagaagaacagtatttggtatctgcgctctgctgaagccagttaccttcggaaaaagagttggtagctcttgatccggcaaacaaaccaccgctggtagcggtggtttttttgtttgcaagcagcagattacgcgcagaaaaaaaggatctcaagaagatcctttgatcttttctacggggtctgacgctcagtggaacgaaaactcacgttaagggattttggtcatgagattatcaaaaaggatcttcacctagatccttttaaattaaaaatgaagttttaaatcaatctaaagtatatatgagtaaacttggtctgacagttaccaatgcttaatcagtgaggcacctatctcagcgatctgtctatttcgttcatccatagttgcctgactccccgtcgtgtagataactacgatacgggagggcttaccatctggccccagtgctgcaatgataccgcgagacccacgctcaccggctccagatttatcagcaataaaccagccagccggaagggccgagcgcagaagtggtcctgcaactttatccgcctccatccagtctattaattgttgccgggaagctagagtaagtagttcgccagttaatagtttgcgcaacgttgttgccattgctacaggcatcgtggtgtcacgctcgtcgtttggtatggcttcattcagctccggttcccaacgatcaaggcgagttacatgatcccccatgttgtgcaaaaaagcggttagctccttcggtcctccgatcgttgtcagaagtaagttggccgcagtgttatcactcatggttatggcagcactgcataattctcttactgtcatgccatccgtaagatgcttttctgtgactggtgagtactcaaccaagtcattctgagaatagtgtatgcggcgaccgagttgctcttgcccggcgtcaatacgggataataccgcgccacatagcagaactttaaaagtgctcatcattggaaaacgttcttcggggcgaaaactctcaaggatcttaccgctgttgagatccagttcgatgtaacccactcgtgcacccaactgatcttcagcatcttttactttcaccagcgtttctgggtgagcaaaaacaggaaggcaaaatgccgcaaaaaagggaataagggcgacacggaaatgttgaatactcatactcttcctttttcaatattattgaagcatttatcagggttattgtctcatgagcggatacatatttgaatgtatttagaaaaataaacaaataggggttccgcgcacatttccccgaaaagtgccacct

SEQ ID NO: 16 - DNA, 461 bp, synthetic construct
  misc_feature 1..461: note = plasmid
  source 1..461: mol_type = other DNA
gagggcccggaaacctggccctgtcttcttgacgagcattcctaggggtctttcccctctcgccaaaggaatgcaaggtctgttgaatgtcgtgaaggaagcagttcctctggaagcttcttgaagacaaacaacgtctgtagcgaccctttgcaggcagcggaaccccccacctggcgacaggtgcctctgcggccaaaagccacgtgtataagatacacctgcaaaggcggcacaaccccagtgccacgttgtgagttggatagttgtggaaagagtcaaatggctcccctcaagcgtattcaacaaggggctgaaggatgcccagaaggtaccccattgtatgggatctgatctggggcctcggtgcacatgctttacatgtgtttagtcgaggttaaaaaacgtctaggccccccgaaccacggggacgtggttttctttgaaaaacacgatgataa